European Patent Application EP 4 328 311 A1, published February 28, 2024. Title: NEGATIVE-STRAND RNA VIRAL VECTOR AND PLANT GENOME EDITING METHOD WITHOUT TRANSFORMATION. Applicant: Zhejiang University. The sequence listing filed with the application follows.

SEQUENCE LISTING (138 sequences)

SEQ ID NO: 1 - DNA, 2967 bp, Tomato spotted wilt virus
  misc_feature: TSWV S genome sequence
agagcaattgtgtcataattttattcttaatcaaacctcacttagaaaatcacaatactgtaataagaacacagtaccaataaccataatgtcttcaagtgtttatgagtcgatcattcagacaaaagcttcagtctggggatcaactgcatctggtaaagctgttgtagattcttactggattcatgaacttggtactggttctccactagttcaaacccagttgtattctgattcaagaagcaaaagtagctttggctatactgcaaaggtggggaatcttccctgtgaagaagaagagattctttctcagcatgtgtatatccctatttttgatgatattgattttagcatcaatattaatgactctgttctggcactatctgtttgctcaaatacagttaatactaacggagtgaaacatcaaggtcatttgaaagttttgtctcctgctcagctccattctattggatctaccatgaacagatctgatattacagaccgattccagctccaagaaaaagacataattcccaatgacagatacattgaagctgcaaacaagggctctttgtcttgtgttaaagagcatacctataaggtcgagatgtgctacaatcaagctttgggcaaagtgaatgttctatcccctaacagaaatgtccatgaatggctgtactgtttcaagccaaatttcaatcaagttgaaagcaacaacagaactgtaaattctcttgcagtgaaatctcttctcatgtcagcagaaaacaacatcatgcctaactctcaggcttttgtaaaagcttccactgattctcatttcaagctgaacctctggctaagagttccaaaggttttgaagcagatttccattcagaaattgttcaaagttgcaggagatgaaacaaacaaaacattttatttatctattgcttgcattccaaaccataacagtgttgagacagctttaaacatttctgttatttgcaagcatcagctcccaatccgtaaatgtcaagctccttttgaattatcaatgatgttttctgatttaaaggagccttacaacattgttcatgatccttcataccctcagaggattgttcatgctctgcttgaaactcacacatcttttgcacaagttctttgcaacaacttgcaagaagatgtgatcatctacactttgaacaactatgagctaactcctggaaagttagatctaggtgaaagaaccttgaattacagtgaagatatctgcaaaaggaaatatttcctttcaaaaacacttgaatgtcttccatctaacacacaaactatgtcttacttagacagtatccaaatcccttcctggaagatagactttgccaggggagaaattaaaatttctccacaatctgtttcagttgcaaaatctttgttaaagcttgatttaagcgggatcaaaaagaaagaatctaagatctcggaagcatatgcttcaggatcaaaataatcttgccgtgtccagcttttcctaattatgttatgtttattttctttctttactcataattatttctctgttttgtcatttcttttgaatttctcctgtttaatagaaaccataaaaataaaaataaaaataaaaataaaatcaaaatgaaacaaaaatcaaaaaatgaaacaaaatcaaacaaaaatcaaaaaatgaaataaaaacaacaaaaaattaaaaaacaaaaacccaaaaagatcccgaaagggacaattttggccaaatttgggttttgttttgttttttgttttttgttttttgtttttattttatttttatttttatttatttattttattttattttattttattttttcttatttttattttatgttttttgttgtttttgttattttgtttattattaagcacaacacacagaaagcaaactttaattaaacacacttattttaaatttaacacactaagcaagcacaagcaataaagataaagaaagctttatatatttataggcttttttataatttaacttacaactgcttttaagcaagttctgcaagttttgtctgttttttaaccccgaacatttcatagaacttgttaagagtttcactgtaatgttccatagcaatacttcctttagcattaggattgctggagctaagtatagcagcatactctttccctttcttcacctgatcttcattcatttcaaatgctttgctttttagcacagtgcaaacttttcctaaggcttccctggtgtcatacttctttggatcgatcccgaggtctttgtattttgcatcctgatatatagccaagacaacactgatcatctcaaagctatcaactgaagcaataagaggtaagctacctcccagcattatggcaagcctcacagactttgcatcatcaagaggtaatccataggcttgaatcagagggtgagaagcaatcttagatttgatagtattgagattctcagaattcccagtttcctcgacaagcctgaccctgatcaagctatcaagccttctgaaggtcatgtcagtggctccaatcctgtctgaagttttctttatagtgattttgccaaaagtaaaatcactttgcttaataaccttcattatactctgacgattcttcaggaatgtcagacatgaaataatgctcatcttcttgatctggtcaaggttttccagacaaaaagtcttgaagttaaatgctaccagattctgatcttcttcaaattcaagatctttgccttgtgtcaacaaagcaacaatgttttccttagtgagcttaaccttagacatgatgatcgtagaagttgttatatgctttgaccgtatgtaattcaaggtgcgaaagtacaactctgtattccgcagtcgtttcttagggttttaatgtgatgatttgtaagactgagtgttaaggtttgaataaaattgacacaattgctct

SEQ ID NO: 2 - DNA, 4770 bp, Tomato spotted wilt virus
  misc_feature: TSWV M genome sequence
agagcaatcagtgcatcagaaatatacctattatacactttgctaagaatcaatcaattacattacacaagctcctctacctcaggctgttgaactcaaaatgttgactttttttggtaataaggggtcttctaagtctgccagaaaggatgaagggcctttagtttcacttgctaaacataacggtaatgttgaagtctcaaaaccatggtcttcttctgatgaaaagcttgctttaaccaaagctatggatacatccaaaggaaagatactgttgaacacagagggaacatcttcctttggaacatatgaatctgattctatcacagaatcagagggttatgatctttctgcaagaatgatagtagatacaaaccaccatatctcaaactggaaaaatgatctttttgtcggcaacgggaagcaaaacgctaataaggtcatcaagatctgtccaacttgggacagcagaaaacaatacatgatgatttccaggattgtgatatgggtctgccccactataccaaaccctacagggaaacttgtggttgctctggtcgatcccaacatgccatctgaaaagcaaatcattctgaagggtcaggggacaataactgatcctatctgttttgttttttatctgaactggtctattccgaaaatgaataacactccagaaaactgctgtcagctgcacttgatgtgcagtcaagaatacaagaagggggtttcttttggtagtgtcatgtattcttggacaaaggagttttgtgattcacccagagctgataaagacaaaagttgcatggtcatacctctaaacagggctattagagctagatctcaagcattcattgaggcttgcaagctgataattcctaaaggaaacagtgagaagcagattaaaaaacagcttaaagaactgagctcaaatcttgagagatcagttgaagaagaggaggaaggggtttctgataatgttgctcagttatcttttgatgaaatatagtacttttaataccacttatttaagcttaaatctctgtttattttgcatttttaaatcaaaaaccaaacaaaaacaaaaataaaaaacaaacaaaaaatcaaaaacaaaaaacaaaaacaaaataaggctgaaaagccaaactttggtccgaagactctttttgttgttttttgtttatttgtatttttgtttgttttttgtttattttatatatatataattcgattaatgtaggaaataggatcaaatttagcttgtgacaagcagcctcagacaaggtgagagaaatccataggtggccttcgtcttgtcattgtatctttcattaacataggggctttgatctcagaaccatcatcatcctctatcttggatctagatttataagatttattcttgacatatcctttacaaattgttgttagaatagaacagaaataaatcacaaggaaaatgaatgcaataagcaatatcactctgatagtatcaaaaaatgagccaaagtaacttgcaatgaaattgaatgggcttttaatataatcccagaagccccatgctgaggaatcagaattatattgttgttcttcatgagcatactcatcattttgatctattatgttctccggttcttctacaataacattattgaccagaacttccacagaaatatccggattgccttctggatacaatgtcattttcttcttatccggattagcagaacaaaacattgttattttgtatttgttagacccttttttaacagccagctgataagtagatagagagcaagcatctatagaaattgcagtagaaaatgtcaaatctgagaaaaattccaaaatgcaagataaaccttgaccgcatagaagacagccattgcaattcaatcttgtcgaagttatggaaggtctcttaggagcaactttaaaaagatcagatggaagatcaacgacaatcttgagtttccctaaactaaaagatttttccaagaaaaaactagagaaatctttgaaactaatgggaatatctgatatttgctctaaaccagatctaaatctgtatgtgtcatatccgcatgttttaatagtgattgattttttccctattgctgcacaatcccaagacatgtcatctccttctagagttttcttagtaaaaataggcactccatcatgagtcaattgtggatgaccaaacattttgacaggatcattcaagtttgcaatatttccagaataaatatggctgtcaggtccatgagctatcagttcacctatagtgataccatcattgtgcagatctgcttgtatatcagcttgaaacaatgcattttcataaggaacctcttcagtaatccttgagcattgacctcctaaaataccagaaatgcaaacatctgccactatagttgattttagcactgaataaattctatatgatttatccatgtcataaatatttcgacagaacccgcatgtagcaccttcattaattgcaaaacaccaagcttcttcacatccccaataagaagttggtgttatacaaaaatcttggaaacctgttaaagcttgattttttctgcaagtgtcacagtttcctgtacaagtggaataaaaatctgtgtgagtgctttggataggagctgttgtgtatttttcagacacttcataatgaattcccacacttttgatataaatcacgaatttttttgctttttctgaggtcttatcatttaacatgaatacagtccctcctcctcctaaaagagattgttctaccatatatctatatttcccatccacaacagaatcaaagatcaatgattgtctgggcagaatgttctctggtatgcttgtttcatttttgtctagagaatctcctgcaatcattccggaaatcttgtctgtacggttataggaatctattataccattcctcaatctcttagcctcatacagaccaatcgatgttaaccccaaagagcttcctgtataatctgaaaacccattatacaaaggtttgttgcgaaataaatctaagtattcgcaacctaatctacattttataagattatcaatagatgggtgtgcaacacaattctggttctctatgcaatcattaggaccttctataacaatgttagtgccaaagatactttctataatcttatcttcttttacattacagtaacattgatctttttcagggcatttttcaaatttgcttgtaaccaaaactggacagcctggaacataaaaacatccactcaaacattgagtagtttgagccatagacatgggcatttgagacaaaatgaccaaacctattaagatttcagtcacaaatttcagcaaactaaagcttagcttagtgttcactattagatggaaccattccatgctagtccacttatgtttgttgtagtcatgatctgtttctttggacagtatgggacactctgaagagtgttcttttgaggctttgcttttgttgcagatgcaaattttagtacactcatgtgtgattatgcacaaattgccacagttagaacatttgaatggaaaatatttccataagcaatttatgagcaacaaaatagggtatgtgatcaagcctataagatcataccagagaaagagaggtttagttgtcttgtttactaaccaccggatagggaaatagatcaacaaagctatcaatattaatcttatccaagagaaattgatgcaggctgtttgcttataaatgctctttgaatatttgattatgcaatctctaactcttttgtttgtttttggtattttagctgatttgtcaccgcacaagagattgtgctcaccatccaacatttcttcagtaaaagtgatgcttgctgatccagaaaaagatatgaccttgtgttccgcattttcaccaggtttttttatcaaataacccatgatcttctcggggctagtgatgctaacagtatagggattggcaaagtttgatttagttattttgcagtctccagataactttacggtttgtaatgatactgttccattagtagggtacgagttataagttataggataattatcttgtgtcaggctttctgaaatgaagaattttgttccaactgaaaaatgccttttgttgtcaagtttggtaatgggaataaccgggactttggagaatctctttggcaaatttaaagaattgtcacatttttctaacccttctgctgaatcagaaacacaggaatatatgacaccattattttccacttgataataaacattataagtggatatcccttttatctcgcattttaatgaagaagcattcaagcagttgttaggaagatccgagacagagattattttttgcgtagttgacccagcaaaaatagggatggttgattcttcttctcgtatctgacgggttccaggagtctgagattctagcattagactagttaaagtctccaagatagccttgcgttgaatcgatgcagcagtgggtacttcattctcagcagaatcatcataaacctcaggatgatctccacgaattatttctactttggcatctgtggctctgaagatcaagaatgccaacaagacagaactcagggcaattgtgaaaagactcacttttaccactagttctagtagttttaaaattctcatcttatacgtctgctcagattataatggttatatgattaatttcaagatgtctggattaaggtttttgtttgcactgattgctct

SEQ ID NO: 3 - DNA, 8913 bp, Tomato spotted wilt virus
  misc_feature: TSWV L genome sequence
agagcaatcaggtacaactaaaacatataatctctccacagccagactttacaaataaattatataagaattccctccagtgaaactataccgggactctatatttatatacactatagatttggttcaccagattgtctttaggctaagtagatctaatctaattctaaataacaataaatttatattctaagttctgtctaatctattattcatgcattgttaggcattacttttaatttaatccgtgtcttcttcttcatcagaatcatcttcgtcaaaggcatcttcttcccctcttagataactaagcaagaaattgtcttcatctgtttcaacaacctcatccaactcacttattttactcaaaataatctctcttgtttgcatgatataatcattgatatcagagtaagtgtatcttccatacaatgttttttctgataagcataatgggtgcctagaaaggaaatttgcgatatctttatagacctctagttttttagttcgcgattgttcatctcttaattgtatcaaagctttcttaactcttccagataagaaatgctccttagacttgctttttgtcagttttagataaccttctaagctgtcagctatctcatttaaaggacaattgacattcttatattccatataaacagttgcataaactttgagtgcaggtacactggaacttaatctgcccagtctgtcagttgaaaatatgtctggtctaaaactattccgcaacaatgtctctatatcaaaactggttccctttatccctccaatcaagaactttatcaactcacttagtaaaagtgtatttgccgggaataaagaccctttcttttttcttttaatcttcatttctttgatcaaaccttcatacatttcttcctcatctagcctcaacacattaaaactggcaagaccttcaaattcttcatcagacctatccatttttagattctctccagatataacaaacccattctcttttagtatctcccttgatagttctgataattttatttctggtaaaaccagtgtcttgaaatcataacttttttccatcaagttattttgcaaatccagatcatgattcaatcttattcttctcccaaatgtggcatatgtcctgctaagaacattcctcaaacttgctaagtttaatatagagtcgttgttgtggcatgtttcgcaagctttaatcagttggatcattcctagcaagttgaattcccctatctctatgtgcttttttgccattagttcgacagcatgcattccagtggctctatagcttttaaatcctgatgcatcatttatcaaagaatatttaagcatgagcagtatttctttgaaaccttctaaatctctagtatactgttttgctttgtcaacaatctctgaaaacagaggactatactcattttcaaagttgtcatgtgttcttaacaagttttcgaatagttctactgtatcattaaacccattttcatcaagatagctatcatattcttccacacttttgcagttttccaaaccttctaagcaggtatcccggatgttcattaagaattcatccatcgtttctctgatatcatcatccacaatctctttgatctgctgtgataagtttccaaaggcttctatgaaagttaaagaagtcataagcctgttttttatggttttgattgtttcagtttcagagtctgcagttttgtacatatcagagaaacattcccctacttcagggagccttaagactagagatttttggctttctataatatcccacacatcggagttcacgttttcatattttatcttcacaactaatttcacattctctagtcttatttgtcttgatgtggcattaacctttacaatcatcttgttgtctgtggtcattctgatgcaggcatctcctggttctaggaaaacaatctgtggttgttttgattttattatgttcactttatcaaacataaatttctgcaataatttctctatactttctctgtatgtgtcaaaaagataatctctttcattcaatatctcaaatggtgtcctcaaagaaactgctacatcttgatcagatgctatcaattgaacataacagcttcttgtcatgatcccgattttgtacatagttccagagatataatttcctgattcgtcttgttcttcagttttcacatatcttacatcacttctcctaatatacctgataacaaaatctaatgttctatgagaacataaacccatgttccacatccagacaatttgtttctggattgtgttcaattcactgttatgtgacagaatcacatttgacactgtgaagccacttgctgttgaattgttaatctttttcattttgtcttctagactcttccatataggtttgctgtctaggcacacattttgcaatatcaaaactatatcctctcttgtaattgttgggaaaagtgactgcaatttatctgatatgtatacagcagtgtccagtattttctctaagttcatatcttgctgagcacttatcacagttctaatagttttgtctaatttataactagctgtagaaacaaaatgataggattcttctttactgtagatggtggataagagagctaatgtgtttgagataaaccctctccctaggttgaatttagaatagaaggggaagcttttcctagtaaagcatgtgttaattgctaaaagcctgttttgtgctgctatcatataattgcatgctttcaccaatctttgacattcgttagaattgctgaaagcctctgtttcgaagctgtctttgcctttaactaaggattttacatcctccatgattaaacctgttccaaacgtgcttgttaaaacattaatgctatcgtctgttagagggatgttttttaaacctaaattttctatataatttgatccatagacagcatgcattaccactaatcccggagagccttcaactacaggtatccacttctcagtctgaaaccacctgaaattgtagttatctcttttcctagattcacaagggtatgcagaatccaatattgggatcagcatgctgaaattaacatccttgatcactagatttacacatgttttaaatgaacaatatgaatctaaatcaaattttagcatttccaagattttcttttccatgttttcttcataagtcatcttcacagtggaagaaatgtctacaaatgttctagcttttgaccttaatactctatccaaagcaagtttctctgtagattggttagataactgattccttttagaagggcttgtgtacatgaacagctgactaagtaaaaaatctctatcattcaatggtgctatcagaattgtttcaggattttttatcattatgtcatgaacagattccatttctaagctagatgcaatcttctcatataactcatctccctctaaaatagcatcctcgtctatctttaagttcttagtacttttatataaatcttcattctttttcaaattagggtaaagttttgaaaaatctttataacttgacatcttgtttaaagcattctcatttataaaattgggcaattttataatctgagttaacatagtttgaaatttcatcccgattgttagaacgtctgaatcttcagacactgatgctttctcaaacagattgataagaaatatcatctttttatctttttcttccagagttcctttttcatactttccttttagctctctgaatctcatctgtagatagctggaagaagagacgctatcttttacttcctctaaactttttttgttcaaaaaatctcttatcacattgtaatagatgatttgatcattcgatgatggacctaatatagacaatggctctataggagaagtcaaccagccccccatgtttgtgggaatctcgtttgactttaaacttactccaagcttcttaaaaattctgatgctatcattcacttcaccaggaagcattgaatagatgcttaatgcttgtacctgtacagccccataagcaaaaggtataacttcattaggacagccttttctcagaagcatcgtaacatgtatacttagtgacattagatcatcaaaataacttatatgtgaagattctgtgcaacaatttgctaaatgtctgcaatagagaggaataattgctccatttacaattctttcagatataaactctacttctgatgaagaagcataactcttttttgggttcaaagttatgcaaaagcttttgaaatgagcttcaatgcttctaaacaacatttctggcagagatgagcttgaaaagtctgttagcattttatcgacctctccactggctatcaatgatgtcgcattatcatcagagtgcacaatccatctagtttggaaatcacagtctttgtagcattctaaagtcttgtgataagctttcattgcacaagagtgataaacagaagacagataatttaaattgccttgtaaccagttcatgctaacagggtatgtgtttgtcgtcaaacctttagtcaaaagtcctatggcagtttcattttgcccgaaagttccttgagcttttcttagattcaaaaaaatatctgttggtatacaaaccttcttcaatttaacatacattagaatacattctatcattaaactagcttcaccagtagttaaaattggatttaatatgatagctaaaacatatttataggtaaggtctgatgccgaccatttcgattgatcagcagacaggaaagccaatcttgacttctttgaattcttgtttaaaatgtcgttgtaagacgtgattgtgtccaaagataatgtagaaagtgcccttattttattgtctccacttatagatatggcttctgatggatcactctgcgcaacatgtttgaatgtgtgctctataaaataaagcatcattttcactttcatactcatcaagtatatttctctgtctgttttggttctctgcattttttcaaaaacagaaactagaaaatctacagacccggtgacatttttagctttggacatgacaaattcaagcatctgcaagaatgtgtgttttttcccttctgtacctttcccaaggttcataacagaatctaagtctatttccatcatgttatgaaactgttttacaaggtcataaagctcctctgatacttttttagactttaaaacagtcacattatttctataatatagttttgttttgagatatgtttctactgttaaaggatggttatttcttataaatttagatgttacggatttccctacagttatcgatccactattaattatctctttaagcttttctacaagatacagtgaattgacacaattatcttcaaaaaattccaccaatctgtttttctcctcattgtaggttcttataagcccttttataatggccaggttatttcctttccaattttctatatcttggatctttgcattctggagacactctattatctcatcagtacttataatgtttgactgcgagcatttttttgaagattttaaagtagatattttataacaagggcttagaaaatcttctttattttctatttctgatctcatcaaacccacattttctatatttcctagatagtaatcagataatgctttcacgttcaaagctccatttatagagaataggtctttgtcatcaaacattgctttcttagggtatatgtcctcaaatatgttgaaacctaactcttttctgaactttagctcccactcagcagggacatttaacaagcttgttagattgtgaacgtgattgtgcaatgatttaggcatcatgtaaatagccaaatagacattattatacaaatcctcaagagtcagtagagttgatcctgttattggacattttatattcaagtctgttatccctcctataatatcattttcatgatctacaacaacgggtttggcatttgtgcttaaattgagatcttccattctgaacaatagctttttgattccattaacgaaatagatatctgccacattggttatatcaggatcaaatttgtctctaatgtactcttttatattagaataatcagacagtggcaaaaaacctgcataccgcatgaagtcaaaaattcccatcctgctgagctttgtcacagttcctatcatgacagatgaaaacacaatatttattaatatctgttttacagtcattgtcatagaaaagacatttactttttctatatctttgtttttcagccatttttccatttcgttagctttctttgaaaattgtgcaaaacatacaggaactttactaggcgttttgaaaaggcttagcagcctcacctgattgagtctctgtggtctcattatataaatgtaattactaccatttcggaaatagctataaatttctttagtataacatatgttaaattgatctgacatgtcttcatccactatatgcaatgctatgtaaggaactcctgatcctccggtgttcattccatctcctttgaatgccaatagcatcatgctcgtatttgctgtggttagtattttgaaactttctttggtcatgtacctgtcagccaccattaaacctttggagaattgcatcatgtcttcagagtaatggtaaatggctaggtcattgcataatttgtttatctttttgcaagtctctaattcagttttcagtactgaatcttgaatgtacaagcattcaggatttttagcataattattgtaaacagatgtgatcttgccttcctctcttatatcaccattatgaagaacaaacaaagagtccttaatcctttcacaccagcttaagctatcctcgttgtcatgtcttatcagttttttcatatgagtcagagatgacatgtctatacttgaataatcatcatttgggtcagcctgcctttcagaggtatcatattccaagcctttagaaatcctctcttttatttcttctttttttagaattctttttttagaactcattcctatattcattactgctaagcctttaaaatagatagttttgttctccctgcctgtctctttcatgcaaaattcatttttgttcctggttaaacacgaaccctgcttattccattctttagatttttttgttctctcaactttaatactcccagtgtttatatctatttcatcctcaagctcctgcttttccatttttgttgtatcacaacttagctctgttaaacacagtctaactaagtttgttatatctcttgctttatttgtgtggttatttatgcaactatatgggctattataaataacccttgaagaacttttgaagctttcccgaaacttgtttataattgcgttgttgtaatctacctctgagctcaattctattttttcaaaacttggggaccaagtcatagaaaagttagttttagtttcagagagatcatttgtaaaacagtttgggtacttttcttcatattcagcagcattctggttaaaagctgtggttatgtcaggtatttctttttcttttttctttttttctctaattctaagcatgattttctcaagatgtttcccatacagagattcccatatttgctgcttctggattaagtggtccttcaaatcagctaaatcaacttttggctctatttttaaattgatacaagagctttggtaccctttaaatttgtcggcgatatgctggtcattcattgtttcaatgtggaaacagaaatttccaaacaaaaaatgtattatttcctctttagttatttcatctgtaacaagtgaatcaattattctttcaatatcttcagaataggctatttcagtaggatttctttctttgtatttgctggtccagtgactaaaaaacacatctttagatccaaaatcatcacctagtattcctctgacttcagatttgatcttttgagtgtttgcataatagtttctcaccactgtgggtgtggttccaactattcgcccaacatgagaaatatttagcaatttggcatttctagcatgctttattctttctccatgcaatgctgatggagaatcttcaaatttctccaaaaccctgctgctagtaacagtgattggcatcccagcaataggtttcaatataactatagaaacgaaaacagggtgatcttccaggaatggctttccattcacttttatatctttgaaagatttccagatatttttgtagtatttctccattgttttagtttctgtcctggcatcgacagatattttccaatcataaatgattaaacaaagctcactgttttttgattctttatatatcacatagttgtcaggtgtggcgttagttgccacatattctttatttattctctcaaactcatcatcagagagcttattaatgcaggactttttgttaagttcatccagatattctctgagcgcatgctctatctccacttcacttctttgtttgggctttattctcaggtgcctggagatcagctctccaaaaatatcatgccttgctaactctgtttctaggtatttttgctcaaatagagaaaccatctcacttaacttcttgacgtctacagttgccatccctttgtttagtccttctccatcagcagtgattttgacaattaactctctcatcgtctcataattttttgcattattattaataatcacatcttctgggatctcatcactatttctcttatgtaaatccaaagctaggtcgtaattagaacctacacaatcctcaatagacaacaataaagtagttccattctctattaatttttgtattttctggatgttcatgtttgcttaaaatcgttgttacctgattgctct

SEQ ID NO: 4 - DNA, 8640 bp, Tomato spotted wilt virus
  misc_feature: RdRP gene sequence
atgaacatccagaaaatacaaaaattaatagagaatggaactactttattgttgtctattgaggattgtgtaggttctaattacgacctagctttggatttacataagagaaatagtgatgagatcccagaagatgtgattattaataataatgcaaaaaattatgagacgatgagagagttaattgtcaaaatcactgctgatggagaaggactaaacaaagggatggcaactgtagacgtcaagaagttaagtgagatggtttctctatttgagcaaaaatacctagaaacagagttagcaaggcatgatatttttggagagctgatctccaggcacctgagaataaagcccaaacaaagaagtgaagtggagatagagcatgcgctcagagaatatctggatgaacttaacaaaaagtcctgcattaataagctctctgatgatgagtttgagagaataaataaagaatatgtggcaactaacgccacacctgacaactatgtgatatataaagaatcaaaaaacagtgagctttgtttaatcatttatgattggaaaatatctgtcgatgccaggacagaaactaaaacaatggagaaatactacaaaaatatctggaaatctttcaaagatataaaagtgaatggaaagccattcctggaagatcaccctgttttcgtttctatagttatattgaaacctattgctgggatgccaatcactgttactagcagcagggttttggagaaatttgaagattctccatcagcattgcatggagaaagaataaagcatgctagaaatgccaaattgctaaatatttctcatgttgggcgaatagttggaaccacacccacagtggtgagaaactattatgcaaacactcaaaagatcaaatctgaagtcagaggaatactaggtgatgattttggatctaaagatgtgttttttagtcactggaccagcaaatacaaagaaagaaatcctactgaaatagcctattctgaagatattgaaagaataattgattcacttgttacagatgaaataactaaagaggaaataatacattttttgtttggaaatttctgtttccacattgaaacaatgaatgaccagcatatcgccgacaaatttaaagggtaccaaagctcttgtatcaatttaaaaatagagccaaaagttgatttagctgatttgaaggaccacttaatccagaagcagcaaatatgggaatctctgtatgggaaacatcttgagaaaatcatgcttagaattagagaaaaaaagaaaaaagaaaaagaaatacctgacataaccacagcttttaaccagaatgctgctgaatatgaagaaaagtacccaaactgttttacaaatgatctctctgaaactaaaactaacttttctatgacttggtccccaagttttgaaaaaatagaattgagctcagaggtagattacaacaacgcaattataaacaagtttcgggaaagcttcaaaagttcttcaagggttatttataatagcccatatagttgcataaataaccacacaaataaagcaagagatataacaaacttagttagactgtgtttaacagagctaagttgtgatacaacaaaaatggaaaagcaggagcttgaggatgaaatagatataaacactgggagtattaaagttgagagaacaaaaaaatctaaagaatggaataagcagggttcgtgtttaaccaggaacaaaaatgaattttgcatgaaagagacaggcagggagaacaaaactatctattttaaaggcttagcagtaatgaatataggaatgagttctaaaaaaagaattctaaaaaaagaagaaataaaagagaggatttctaaaggcttggaatatgatacctctgaaaggcaggctgacccaaatgatgattattcaagtatagacatgtcatctctgactcatatgaaaaaactgataagacatgacaacgaggatagcttaagctggtgtgaaaggattaaggactctttgtttgttcttcataatggtgatataagagaggaaggcaagatcacatctgtttacaataattatgctaaaaatcctgaatgcttgtacattcaagattcagtactgaaaactgaattagagacttgcaaaaagataaacaaattatgcaatgacctagccatttaccattactctgaagacatgatgcaattctccaaaggtttaatggtggctgacaggtacatgaccaaagaaagtttcaaaatactaaccacagcaaatacgagcatgatgctattggcattcaaaggagatggaatgaacaccggaggatcaggagttccttacatagcattgcatatagtggatgaagacatgtcagatcaatttaacatatgttatactaaagaaatttatagctatttccgaaatggtagtaattacatttatataatgagaccacagagactcaatcaggtgaggctgctaagccttttcaaaacgcctagtaaagttcctgtatgttttgcacaattttcaaagaaagctaacgaaatggaaaaatggctgaaaaacaaagatatagaaaaagtaaatgtcttttctatgacaatgactgtaaaacagatattaataaatattgtgttttcatctgtcatgataggaactgtgacaaagctcagcaggatgggaatttttgacttcatgcggtatgcaggttttttgccactgtctgattattctaatataaaagagtacattagagacaaatttgatcctgatataaccaatgtggcagatatctatttcgttaatggaatcaaaaagctattgttcagaatggaagatctcaatttaagcacaaatgccaaacccgttgttgtagatcatgaaaatgatattataggagggataacagacttgaatataaaatgtccaataacaggatcaactctactgactcttgaggatttgtataataatgtctatttggctatttacatgatgcctaaatcattgcacaatcacgttcacaatctaacaagcttgttaaatgtccctgctgagtgggagctaaagttcagaaaagagttaggtttcaacatatttgaggacatataccctaagaaagcaatgtttgatgacaaagacctattctctataaatggagctttgaacgtgaaagcattatctgattactatctaggaaatatagaaaatgtgggtttgatgagatcagaaatagaaaataaagaagattttctaagcccttgttataaaatatctactttaaaatcttcaaaaaaatgctcgcagtcaaacattataagtactgatgagataatagagtgtctccagaatgcaaagatccaagatatagaaaattggaaaggaaataacctggccattataaaagggcttataagaacctacaatgaggagaaaaacagattggtggaattttttgaagataattgtgtcaattcactgtatcttgtagaaaagcttaaagagataattaatagtggatcgataactgtagggaaatccgtaacatctaaatttataagaaataaccatcctttaacagtagaaacatatctcaaaacaaaactatattatagaaataatgtgactgttttaaagtctaaaaaagtatcagaggagctttatgaccttgtaaaacagtttcataacatgatggaaatagacttagattctgttatgaaccttgggaaaggtacagaagggaaaaaacacacattcttgcagatgcttgaatttgtcatgtccaaagctaaaaatgtcaccgggtctgtagattttctagtttctgtttttgaaaaaatgcagagaaccaaaacagacagagaaatatacttgatgagtatgaaagtgaaaatgatgctttattttatagagcacacattcaaacatgttgcgcagagtgatccatcagaagccatatctataagtggagacaataaaataagggcactttctacattatctttggacacaatcacgtcttacaacgacattttaaacaagaattcaaagaagtcaagattggctttcctgtctgctgatcaatcgaaatggtcggcatcagaccttacctataaatatgttttagctatcatattaaatccaattttaactactggtgaagctagtttaatgatagaatgtattctaatgtatgttaaattgaagaaggtttgtataccaacagatatttttttgaatctaagaaaagctcaaggaactttcgggcaaaatgaaactgccataggacttttgactaaaggtttgacgacaaacacataccctgttagcatgaactggttacaaggcaatttaaattatctgtcttctgtttatcactcttgtgcaatgaaagcttatcacaagactttagaatgctacaaagactgtgatttccaaactagatggattgtgcactctgatgataatgcgacatcattgatagccagtggagaggtcgataaaatgctaacagacttttcaagctcatctctgccagaaatgttgtttagaagcattgaagctcatttcaaaagcttttgcataactttgaacccaaaaaagagttatgcttcttcatcagaagtagagtttatatctgaaagaattgtaaatggagcaattattcctctctattgcagacatttagcaaattgttgcacagaatcttcacatataagttattttgatgatctaatgtcactaagtatacatgttacgatgcttctgagaaaaggctgtcctaatgaagttataccttttgcttatggggctgtacaggtacaagcattaagcatctattcaatgcttcctggtgaagtgaatgatagcatcagaatttttaagaagcttggagtaagtttaaagtcaaacgagattcccacaaacatggggggctggttgacttctcctatagagccattgtctatattaggtccatcatcgaatgatcaaatcatctattacaatgtgataagagattttttgaacaaaaaaagtttagaggaagtaaaagatagcgtctcttcttccagctatctacagatgagattcagagagctaaaaggaaagtatgaaaaaggaactctggaagaaaaagataaaaagatgatatttcttatcaatctgtttgagaaagcatcagtgtctgaagattcagacgttctaacaatcgggatgaaatttcaaactatgttaactcagattataaaattgcccaattttataaatgagaatgctttaaacaagatgtcaagttataaagatttttcaaaactttaccctaatttgaaaaagaatgaagatttatataaaagtactaagaacttaaagatagacgaggatgctattttagagggagatgagttatatgagaagattgcatctagcttagaaatggaatctgttcatgacataatgataaaaaatcctgaaacaattctgatagcaccattgaatgatagagattttttacttagtcagctgttcatgtacacaagcccttctaaaaggaatcagttatctaaccaatctacagagaaacttgctttggatagagtattaaggtcaaaagctagaacatttgtagacatttcttccactgtgaagatgacttatgaagaaaacatggaaaagaaaatcttggaaatgctaaaatttgatttagattcatattgttcatttaaaacatgtgtaaatctagtgatcaaggatgttaatttcagcatgctgatcccaatattggattctgcatacccttgtgaatctaggaaaagagataactacaatttcaggtggtttcagactgagaagtggatacctgtagttgaaggctctccgggattagtggtaatgcatgctgtctatggatcaaattatatagaaaatttaggtttaaaaaacatccctctaacagacgatagcattaatgttttaacaagcacgtttggaacaggtttaatcatggaggatgtaaaatccttagttaaaggcaaagacagcttcgaaacagaggctttcagcaattctaacgaatgtcaaagattggtgaaagcatgcaattatatgatagcagcacaaaacaggcttttagcaattaacacatgctttactaggaaaagcttccccttctattctaaattcaacctagggagagggtttatctcaaacacattagctctcttatccaccatctacagtaaagaagaatcctatcattttgtttctacagctagttataaattagacaaaactattagaactgtgataagtgctcagcaagatatgaacttagagaaaatactggacactgctgtatacatatcagataaattgcagtcacttttcccaacaattacaagagaggatatagttttgatattgcaaaatgtgtgcctagacagcaaacctatatggaagagtctagaagacaaaatgaaaaagattaacaattcaacagcaagtggcttcacagtgtcaaatgtgattctgtcacataacagtgaattgaacacaatccagaaacaaattgtctggatgtggaacatgggtttatgttctcatagaacattagattttgttatcaggtatattaggagaagtgatgtaagatatgtgaaaactgaagaacaagacgaatcaggaaattatatctctggaactatgtacaaaatcgggatcatgacaagaagctgttatgttcaattgatagcatctgatcaagatgtagcagtttctttgaggacaccatttgagatattgaatgaaagagattatctttttgacacatacagagaaagtatagagaaattattgcagaaatttatgtttgataaagtgaacataataaaatcaaaacaaccacagattgttttcctagaaccaggagatgcctgcatcagaatgaccacagacaacaagatgattgtaaaggttaatgccacatcaagacaaataagactagagaatgtgaaattagttgtgaagataaaatatgaaaacgtgaactccgatgtgtgggatattatagaaagccaaaaatctctagtcttaaggctccctgaagtaggggaatgtttctctgatatgtacaaaactgcagactctgaaactgaaacaatcaaaaccataaaaaacaggcttatgacttctttaactttcatagaagcctttggaaacttatcacagcagatcaaagagattgtggatgatgatatcagagaaacgatggatgaattcttaatgaacatccgggatacctgcttagaaggtttggaaaactgcaaaagtgtggaagaatatgatagctatcttgatgaaaatgggtttaatgatacagtagaactattcgaaaacttgttaagaacacatgacaactttgaaaatgagtatagtcctctgttttcagagattgttgacaaagcaaaacagtatactagagatttagaaggtttcaaagaaatactgctcatgcttaaatattctttgataaatgatgcatcaggatttaaaagctatagagccactggaatgcatgctgtcgaactaatggcaaaaaagcacatagagataggggaattcaacttgctaggaatgatccaactgattaaagcttgcgaaacatgccacaacaacgactctatattaaacttagcaagtttgaggaatgttcttagcaggacatatgccacatttgggagaagaataagattgaatcatgatctggatttgcaaaataacttgatggaaaaaagttatgatttcaagacactggttttaccagaaataaaattatcagaactatcaagggagatactaaaagagaatgggtttgttatatctggagagaatctaaaaatggataggtctgatgaagaatttgaaggtcttgccagttttaatgtgttgaggctagatgaggaagaaatgtatgaaggtttgatcaaagaaatgaagattaaaagaaaaaagaaagggtctttattcccggcaaatacacttttactaagtgagttgataaagttcttgattggagggataaagggaaccagttttgatatagagacattgttgcggaatagttttagaccagacatattttcaactgacagactgggcagattaagttccagtgtacctgcactcaaagtttatgcaactgtttatatggaatataagaatgtcaattgtcctttaaatgagatagctgacagcttagaaggttatctaaaactgacaaaaagcaagtctaaggagcatttcttatctggaagagttaagaaagctttgatacaattaagagatgaacaatcgcgaactaaaaaactagaggtctataaagatatcgcaaatttcctttctaggcacccattatgcttatcagaaaaaacattgtatggaagatacacttactctgatatcaatgattatatcatgcaaacaagagagattattttgagtaaaataagtgagttggatgaggttgttgaaacagatgaagacaatttcttgcttagttatctaagaggggaagaagatgcctttgacgaagatgattctgatgaagaagaagacacggattaa

SEQ ID NO: 5 - DNA, 8640 bp, Artificial Sequence
  Codon-optimized RdRp gene sequence
atgaacatccagaaaatccagaagctgattgagaacggaactacacttctgttgtctattgaggattgcgtgggcagcaactacgatcttgctcttgatctccacaagcggaactccgatgagattcctgaggacgtgatcatcaacaacaacgccaagaactacgagactatgcgtgagctgatcgtgaagatcactgctgatggtgagggtctgaacaaaggtatggctaccgtggacgtgaagaaactgtctgagatggtgtctctgttcgagcagaagtaccttgagactgagcttgctaggcacgatatcttcggcgagcttatttctaggcacctgaggatcaagccgaagcagaggtcagaggtcgagatcgagcacgccctgagggagtacctggacgagctcaacaagaaatcctgcatcaacaagctgagcgacgacgagttcgagcggatcaacaaagaatatgttgcaaccaatgctacaccagacaattacgttatctacaaggaaagtaagaatagcgagctttgcctgatcatctacgactggaagatttctgtggatgccaggactgagactaagaccatggaaaagtactacaagaacatctggaagtccttcaaggacatcaaagtcaacggcaagcccttcctggaggaccacccggtcttcgtgagcatcgtgatcctgaagcctattgctggcatgcctattaccgtgacctctagcagagtgctcgagaagtttgaggactctccttctgcacttcacggcgagaggattaagcacgctaggaacgctaagctgctgaacatttctcacgtgggtcagatcgtgggtactactcctactgtggtgaggaactactacgctaacacccagaagatcaagtccgaggttagaggtatcctgggtgacgatttcggcagcaaggacgtgttcttctctcactggacctccaagtacaaagagcggaaccctaccgagatcgcttactctgaggatatcgagcgtatcatcgacagccttgtgaccgacgagatcaccaaagaagagattatccacttcctgttcggcaacttctgcttccacatcgagactatgaacgaccagcacattgccgacaagttcaagggctatcagtcctcttgcatcaacctgaagatcgagcctaaggtggacctggctgatcttaaggatcacctgattcagaagcagcagatttgggagagcctgtacggaaagcacctcgagaagattatgctgcggatccgtgaaaagaagaagaaagagaaagagatcccggacatcaccaccgccttcaatcaaaatgctgccgagtacgaagagaagtacccgaactgcttcaccaacgacctgtcagagacaaagaccaacttctctatgacctggtcaccgagcttcgagaaaatcgagctgtctagcgaggtggactacaacaatgccattatcaacaagttccgtgagagcttcaagtccagcagcagagtgatctacaacagcccttacagctgcattaacaaccagaccaacaaggcccgggatatcactaaccttgtgaggctttgcctgaccgagctttcttgcgataccaccaagatggaaaagcaagagcttgaggacgagatcgacatcaacaccggtagcattaaggtcgagcggaccaagaaaagcaaagagtggaacaagcagggctcctgccttactaggaacaagaacgagttctgcatgaaggaaaccggccgagagaacaagaccatctacttcaagggtcttgccgtgatgaacatcggcatgtcctctaagaagcggattctgaagaaagaggaaatcaaagagaggatcagcaagggcctcgagtacgatacttctgagagacaggctgatccgaacgacgactacagcagcatcgatatgtcatcactgacccatatgaagaagctcatccggcacgataacgaggactcactttcttggtgcgagcgaatcaaggacagcttgttcgtgcttcacaacggcgatatcagagaagagggcaagatcaccagcgtgtacaacaattacgctaagaatcccgagtgcctgtacatccaggattctgtgcttaagaccgagctggaaacctgcaagaaaatcaacaaactgtgcaacgatctggccatctaccactacagcgaggacatgatgcagttctccaagggtttgatggtggccgatcggtacatgaccaaagagtctttcaagatcctgaccaccgccaataccagcatgatgctgcttgctttcaaaggcgacggcatgaacaccggcggtagcggcgtgccttacattgccctgcacatcgtggacgaggatatgtccgaccagttcaacatctgctacaccaaagagatctacagctacttccgcaacggctccaactacatctacatcatgaggccgcagaggctcaaccaggtgaggcttctttcactgttcaagacaccttctaaggtgccagtttgcttcgcccagttcagcaagaaggccaacgagatggaaaagtggctgaagaacaaggacattgagaaggtcaacgtgttcagcatgaccatgaccgtgaagcagatcctgatcaacatcgtgttctccagcgtgatgattggcaccgtgactaagctttctcggatgggcatcttcgacttcatgaggtacgctggtttcttgccgctgtccgactactccaacatcaaagagtacatccgggacaagttcgatccagatattaccaatgtggccgatatctacttcgtgaacgggatcaagaaactgctgttccggatggaagatttgaacctgagcaccaacgcaaagcctgttgtggtggatcacgagaacgatatcatcggtggcatcaccgacctgaacatcaagtgccctattactggttctaccctgctgaccctcgaggacctgtacaacaacgtgtacctcgccatctacatgatgccgaagtctctgcataaccacgtgcacaaccttaccagcctgcttaatgttcctgctgagtgggagctgaagttccggaaagagcttggcttcaacattttcgaggacatctacccgaagaaagccatgttcgatgacaaggacctcttcagcattaacggcgctcttaacgtgaaggccctgagcgattactacctgggtaacatcgagaatgtgggcctgatgaggtccgagattgagaacaaagaggacttcctgtctccgtgctacaagatctctaccctgaagtccagtaagaagtgcagccagagcaacatcatcagcactgatgagatcattgagtgcctgcagaacgcaaagattcaggacatcgaaaactggaagggcaacaacctggctattatcaagggcctgatccggacctacaacgaggaaaagaatcggctggttgagttcttcgaggataactgcgtgaacagcctgtacctggtcgagaagcttaaagagatcattaacagcggcagcatcaccgtgggaaagtctgtgactagcaagttcatccgtaacaatcacccgctgaccgtggaaacctacctcaagactaagctgtactatcggaacaacgtgaccgtgctgaagtctaagaaggtgagcgaggaactgtacgacctcgttaagcagttccacaacatgatggaaatcgacctggactctgtgatgaaccttggaaagggtactgagggaaagaagcacaccttcttgcagatgcttgagttcgtgatgagcaaggccaagaatgtgaccggttctgtggatttcctcgtgagcgtgttcgaaaagatgcagaggaccaagaccgaccgtgagatctacctgatgagcatgaaggtgaagatgatgctgtacttcatcgagcataccttcaagcacgtggcccagtctgatccttctgaggctattagcatcagcggcgacaacaagattagggctctgtctacccttagcctggacaccattaccagctacaacgacatcctcaacaagaatagcaagaagtctcggctggctttcctgagcgctgatcaatctaagtggtccgcttctgacctgacctacaagtatgtgctggccatcattctgaacccgattcttactactggcgaggcctctcttatgatcgagtgcattctgatgtatgtgaagctgaagaaagtgtgcatcccgaccgacattttcttgaaccttaggaaggctcagggcaccttcggtcaaaacgaaaccgctattggtctgctgaccaagggacttaccaccaacacttacccggtgtctatgaactggctgcagggtaacctgaactacctctcttctgtgtaccactcctgcgctatgaaggcttaccacaagactctcgagtgctataaggactgcgactttcagacccggtggatcgttcactctgatgataacgcaaccagcctgatcgcttcaggtgaggttgacaagatgctgaccgacttctcctcttcatctctgcctgagatgctgttcagatccatcgaggctcacttcaagtctttctgcatcacactcaacccaaagaagtcatacgccagctcaagcgaggtcgagttcatttctgagaggattgtgaacggcgctatcatcccactttactgcagacatcttgctaactgctgcaccgagtcctctcacatctcctacttcgatgacctgatgtccctgtctatccacgtgaccatgttgctgagaaagggctgccctaatgaggttatccctttcgcttacggtgctgtgcaagtgcaggctctctctatctactctatgctgcctggtgaggtgaatgatagcattcggatctttaagaagctgggagtcagccttaagtctaatgagattcctactaacatgggaggttggctgacctctccaattgagcctttgtctattctgggtccaagcagcaacgaccagatcatctactacaacgtcatccgcgatttcctgaacaagaaatcgctggaggaggtgaaagactccgtgtcgtcctcatcctacctgcagatgaggttcagggaactcaagggcaagtacgagaagggtactctggaagagaaggacaagaaaatgatcttccttatcaacctcttcgagaaggccagcgtgtccgaggatagtgatgtgcttaccatcgggatgaagttccagaccatgctgacccagatcatcaagctgcccaacttcatcaacgagaacgccttgaacaagatgagcagctacaaggacttctccaagctgtaccctaacctcaagaagaacgaggatctgtacaagtccaccaagaacctcaaaatcgacgaggacgctatcctcgagggagatgagctttatgagaagatcgccagcagcctcgagatggaatctgtgcacgacatcatgatcaagaacccggaaaccattctgatcgctccgctgaacgatagggactttctgctgtctcagctgttcatgtacacctctccgtctaagaggaaccagctgtctaatcagtctaccgagaagctggctcttgatagggtgttgagatctaaggctaggaccttcgtggacatctcctctaccgttaagatgacctatgaagagaacatggagaagaagatcttggagatgctcaagttcgatctcgacagctactgcagcttcaagacttgcgtgaacctcgtgatcaaggatgtgaacttctccatgcttatcccgatcctcgactctgcttatccttgcgagtctaggaagcgggacaactacaacttccgttggttccagactgagaagtggatccctgttgttgagggttctcctggacttgttgtgatgcatgctgtgtacgggtctaactatatcgagaacctcggccttaagaacatcccgcttaccgacgactctatcaacgtgctgacttctaccttcggcaccggtctgattatggaagatgtcaagagcctggtgaagggcaaagactcatttgagacagaggccttcagcaactctaacgagtgccagagacttgtgaaggcctgcaactacatgatcgctgctcagaacaggctcctggctatcaatacctgctttacccggaagtctttcccgttctactccaagttcaatcttggcagaggcttcatcagcaacacccttgctttgctgtccaccatctacagcaaagaggaatcctaccacttcgtgtccaccgcctcttacaagctggataagactatccggaccgtgatctctgcacagcaggatatgaacctggaaaagatcctggataccgccgtgtacatcagcgacaagcttcagtctttgttcccgaccatcaccagagaggacatcgttctcattctccagaacgtgtgcctggactccaagcctatttggcagtctttggaggacaagatgaagaagattaacaacagcaccgccagcggcttcaccgtgtctaatgtgattctgagccacaactccgagctgaacaccatccagaaacagatcgtgtggatgtggaacatgggcctttgctctcataggaccctggatttcgtgatccgttacatcaggcggtccgatgtgagatacgtcaagactgaggaacaggacgagagcgggaactacattagcggaaccatgtacaagattggcatcatgacccggtcttgctacgtgcagttgatcgcatcagatcaggatgtggctgtgtctcttaggacacctttcgagattctcaacgagagggattacctgttcgacacctaccgtgagtccatcgaaaagctgctgcaaaagttcatgttcgacaaggtcaacattatcaagtctaagcagccgcagattgtgttcctcgagccaggagatgcttgcattaggatgaccaccgacaacaaaatgatcgtcaaggttaacgccaccagcaggcagattaggcttgagaacgttaagctggtggtgaagattaagtatgagaacgtgaactccgacgtgtgggacatcattgagagccagaagtctctcgttctccggcttcctgaagttggtgagtgcttcagcgacatgtataagaccgctgacagcgagactgagacaatcaagactatcaagaaccggctgatgacctctctgaccttcattgaggctttcggcaacctcagccagcagatcaaagaaatcgtggacgatgacatcagggaaaccatggacgagttcctcatgaacatccgtgatacctgccttgagggtcttgagaattgcaagagcgtggaagagtacgactcctaccttgatgagaacgggttcaacgataccgtcgagctgttcgagaatcttctgaggacccacgacaacttcgagaacgagtactctccactgttcagcgagatcgtggataaggctaagcagtacaccagggatctcgagggctttaaagaaatcctgctgatgctgaagtactctctgatcaacgacgcctccgggttcaagtcatatagagctactggtatgcacgccgttgagctgatggctaagaaacacattgagatcggcgagttcaacctgctgggtatgattcagcttatcaaggcttgcgagacttgccacaacaacgactccattctcaacctggccagccttaggaatgtgctgtctaggacttacgctactttcggcaggcggatcaggttgaatcacgatctggatctgcagaacaaccttatggaaaagagctacgacttcaagaccttggtgctccccgagattaagctctctgagctgagcagggaaatcctgaaagagaacggcttcgttatctccggcgagaaccttaagatggacaggtccgatgaagagttcgagggactcgcttcattcaatgtgcttaggttggacgaggaagagatgtacgagggactgatcaaagagatgaagatcaagcggaagaagaagggctctctgttccctgctaataccctgcttctgtccgagttgatcaagttcctgatcggcggtattaagggcaccagcttcgatattgagactctgctccggaactcattcaggccggatatcttctctaccgacaggcttggtaggctctcttcttctgtgcctgctcttaaggtgtacgccactgtgtacatggagtacaagaacgtcaactgccctctgaacgagatcgccgattctcttgagggttacctgaagctcaccaagtccaagagcaaagaacacttcttgagcggcagggtgaagaaggctcttattcagttgagggacgagcagtccaggaccaagaaactcgaggtctacaaggatatcgccaacttccttagcaggcaccctctttgcctgtctgaaaagacactgtacggccggtacacctacagcgatatcaacgattacatcatgcagacccgggaaatcatcctctctaagatctccgagttggatgaggtggtggaaactgacgaggacaacttcctgctctcttaccttagaggcgaagaggatgctttcgatgaggacgattctgatgaggaagaggacaccgattag

SEQ ID NO: 6 - DNA, 3408 bp, Tomato spotted wilt virus
  misc_feature: GP gene sequence
atgagaattttaaaactactagaactagtggtaaaagtgagtcttttcacaattgccctgagttctgtcttgttggcattcttgatcttcagagccacagatgccaaagtagaaataattcgtggagatcatcctgaggtttatgatgattctgctgagaatgaagtacccactgctgcatcgattcaacgcaaggctatcttggagactttaactagtctaatgctagaatctcagactcctggaacccgtcagatacgagaagaagaatcaaccatccctatttttgctgggtcaactacgcaaaaaataatctctgtctcggatcttcctaacaactgcttgaatgcttcttcattaaaatgcgagataaaagggatatccacttataatgtttattatcaagtggaaaataatggtgtcatatattcctgtgtttctgattcagcagaagggttagaaaaatgtgacaattctttaaatttgccaaagagattctccaaagtcccggttattcccattaccaaacttgacaacaaaaggcatttttcagttggaacaaaattcttcatttcagaaagcctgacacaagataattatcctataacttataactcgtaccctactaatggaacagtatcattacaaaccgtaaagttatctggagactgcaaaataactaaatcaaactttgccaatccctatactgttagcatcactagccccgagaagatcatgggttatttgataaaaaaacctggtgaaaatgcggaacacaaggtcatatctttttctggatcagcaagcatcacttttactgaagaaatgttggatggtgagcacaatctcttgtgcggtgacaaatcagctaaaataccaaaaacaaacaaaagagttagagattgcataatcaaatattcaaagagcatttataagcaaacagcctgcatcaatttctcttggataagattaatattgatagctttgttgatctatttccctatccggtggttagtaaacaagacaactaaacctctctttctctggtatgatcttataggcttgatcacataccctattttgttgctcataaattgcttatggaaatattttccattcaaatgttctaactgtggcaatttgtgcataatcacacatgagtgtactaaaatttgcatctgcaacaaaagcaaagcctcaaaagaacactcttcagagtgtcccatactgtccaaagaaacagatcatgactacaacaaacataagtggactagcatggaatggttccatctaatagtgaacactaagctaagctttagtttgctgaaatttgtgactgaaatcttaataggtttggtcattttgtctcaaatgcccatgtctatggctcaaactactcaatgtttgagtggatgtttttatgttccaggctgtccagttttggttacaagcaaatttgaaaaatgccctgaaaaagatcaatgttactgtaatgtaaaagaagataagattatagaaagtatctttggcactaacattgttatagaaggtcctaatgattgcatagagaaccagaattgtgttgcacacccatctattgataatcttataaaatgtagattaggttgcgaatacttagatttatttcgcaacaaacctttgtataatgggttttcagattatacaggaagctctttggggttaacatcgattggtctgtatgaggctaagagattgaggaatggtataatagattcctataaccgtacagacaagatttccggaatgattgcaggagattctctagacaaaaatgaaacaagcataccagagaacattctgcccagacaatcattgatctttgattctgttgtggatgggaaatatagatatatggtagaacaatctcttttaggaggaggagggactgtattcatgttaaatgataagacctcagaaaaagcaaaaaaattcgtgatttatatcaaaagtgtgggaattcattatgaagtgtctgaaaaatacacaacagctcctatccaaagcactcacacagatttttattccacttgtacaggaaactgtgacacttgcagaaaaaatcaagctttaacaggtttccaagatttttgtataacaccaacttcttattggggatgtgaagaagcttggtgttttgcaattaatgaaggtgctacatgcgggttctgtcgaaatatttatgacatggataaatcatatagaatttattcagtgctaaaatcaactatagtggcagatgtttgcatttctggtattttaggaggtcaatgctcaaggattactgaagaggttccttatgaaaatgcattgtttcaagctgatatacaagcagatctgcacaatgatggtatcactataggtgaactgatagctcatggacctgacagccatatttattctggaaatattgcaaacttgaatgatcctgtcaaaatgtttggtcatccacaattgactcatgatggagtgcctatttttactaagaaaactctagaaggagatgacatgtcttgggattgtgcagcaatagggaaaaaatcaatcactattaaaacatgcggatatgacacatacagatttagatctggtttagagcaaatatcagatattcccattagtttcaaagatttctctagttttttcttggaaaaatcttttagtttagggaaactcaagattgtcgttgatcttccatctgatctttttaaagttgctcctaagagaccttccataacttcgacaagattgaattgcaatggctgtcttctatgcggtcaaggtttatcttgcattttggaatttttctcagatttgacattttctactgcaatttctatagatgcttgctctctatctacttatcagctggctgttaaaaaagggtctaacaaatacaaaataacaatgttttgttctgctaatccggataagaagaaaatgacattgtatccagaaggcaatccggatatttctgtggaagttctggtcaataatgttattgtagaagaaccggagaacataatagatcaaaatgatgagtatgctcatgaagaacaacaatataattctgattcctcagcatggggcttctgggattatattaaaagcccattcaatttcattgcaagttactttggctcattttttgatactatcagagtgatattgcttattgcattcattttccttgtgatttatttctgttctattctaacaacaatttgtaaaggatatgtcaagaataaatcttataaatctagatccaagatagaggatgatgatggttctgagatcaaagcccctatgttaatgaaagatacaatgacaagacgaaggccacctatggatttctctcaccttgtctga

SEQ ID NO: 7 - DNA, 1404 bp, Tomato spotted wilt virus
  misc_feature: NSs sequence
atgtcttcaagtgtttatgagtcgatcattcagacaaaagcttcagtctggggatcaactgcatctggtaaagctgttgtagattcttactggattcatgaacttggtactggttctccactagttcaaacccagttgtattctgattcaagaagcaaaagtagctttggctatactgcaaaggtggggaatcttccctgtgaagaagaagagattctttctcagcatgtgtatatccctatttttgatgatattgattttagcatcaatattaatgactctgttctggcactatctgtttgctcaaatacagttaatactaacggagtgaaacatcaaggtcatttgaaagttttgtctcctgctcagctccattctattggatctaccatgaacagatctgatattacagaccgattccagctccaagaaaaagacataattcccaatgacagatacattgaagctgcaaacaagggctctttgtcttgtgttaaagagcatacctataaggtcgagatgtgctacaatcaagctttgggcaaagtgaatgttctatcccctaacagaaatgtccatgaatggctgtactgtttcaagccaaatttcaatcaagttgaaagcaacaacagaactgtaaattctcttgcagtgaaatctcttctcatgtcagcagaaaacaacatcatgcctaactctcaggcttttgtaaaagcttccactgattctcatttcaagctgaacctctggctaagagttccaaaggttttgaagcagatttccattcagaaattgttcaaagttgcaggagatgaaacaaacaaaacattttatttatctattgcttgcattccaaaccataacagtgttgagacagctttaaacatttctgttatttgcaagcatcagctcccaatccgtaaatgtcaagctccttttgaattatcaatgatgttttctgatttaaaggagccttacaacattgttcatgatccttcataccctcagaggattgttcatgctctgcttgaaactcacacatcttttgcacaagttctttgcaacaacttgcaagaagatgtgatcatctacactttgaacaactatgagctaactcctggaaagttagatctaggtgaaagaaccttgaattacagtgaagatatctgcaaaaggaaatatttcctttcaaaaacacttgaatgtcttccatctaacacacaaactatgtcttacttagacagtatccaaatcccttcctggaagatagactttgccaggggagaaattaaaatttctccacaatctgtttcagttgcaaaatctttgttaaagcttgatttaagcgggatcaaaaagaaagaatctaagatctcggaagcatatgcttcaggatcaaaataa

SEQ ID NO: 8 - DNA, 909 bp, Tomato spotted wilt virus
  misc_feature: NSm sequence
atgttgactttttttggtaataaggggtcttctaagtctgccagaaaggatgaagggcctttagtttcacttgctaaacataacggtaatgttgaagtctcaaaaccatggtcttcttctgatgaaaagcttgctttaaccaaagctatggatacatccaaaggaaagatactgttgaacacagagggaacatcttcctttggaacatatgaatctgattctatcacagaatcagagggttatgatctttctgcaagaatgatagtagatacaaaccaccatatctcaaactggaaaaatgatctttttgtcggcaacgggaagcaaaacgctaataaggtcatcaagatctgtccaacttgggacagcagaaaacaatacatgatgatttccaggattgtgatatgggtctgccccactataccaaaccctacagggaaacttgtggttgctctggtcgatcccaacatgccatctgaaaagcaaatcattctgaagggtcaggggacaataactgatcctatctgttttgttttttatctgaactggtctattccgaaaatgaataacactccagaaaactgctgtcagctgcacttgatgtgcagtcaagaatacaagaagggggtttcttttggtagtgtcatgtattcttggacaaaggagttttgtgattcacccagagctgataaagacaaaagttgcatggtcatacctctaaacagggctattagagctagatctcaagcattcattgaggcttgcaagctgataattcctaaaggaaacagtgagaagcagattaaaaaacagcttaaagaactgagctcaaatcttgagagatcagttgaagaagaggaggaaggggtttctgataatgttgctcagttatcttttgatgaaatatag

SEQ ID NO: 9 - DNA, 767 bp, Artificial Sequence
  35S promoter sequence
aagcttgcatgcctgcagtcaacatggtggagcacgacactctcgtctactccaagaatatcaaagatacagtctcagaagaccagagggctattgagacttttcaacaaagggtaatatcgggaaacctcctcggattccattgcccagctatctgtcacttcatcgaaaggacagtagaaaaggaagatggcttctacaaatgccatcattgcgataaaggaaaggctatcgttcaaagaatgcctctaccgacagtggtcccaaagatggaccccccacccacgaggaacatcgtggaaaaagaagacgttccaaccacgtcttcaaagcaagtggattgatgtgataacatggtggagcacgacactctcgtctactccaagaatatcaaagatacagtctcagaagaccagagggctattgagactttcaacaaagggtaatatcgggaaacctcctcggattccattgcccagctatctgtcacttcatcgaaaggacagtagaaaaggaagatggcttctacaaatgccatcattgcgataaaggaaaggctatcgttcaagaatgcctctaccgacagtggtcccaaagatggacccccacccacgaggaacatcgtggaaaaagaagacgttccaaccacgtcttcaaagcaagtggattgatgtgatatctccactgacgtaagggatgacgcacaatcccactatccttcgcaagacccttcctctatataaggaagttcatttcatttggagagg

SEQ ID NO: 10 - DNA, 3888 bp, Artificial Sequence
  Rice codon-optimized LbCas12a gene sequence
atggattacaaggatgacgacgataagatggattataaagacgatgacgataagatggattacaaggatgacgacgataagcccgggggatcctctagagtcgacatggctcctaagaagaagcggaaggttggtattcacggggtgcctgcggcttcaaagctcgagaaattcaccaactgttattcgttgagcaaaacactgcggtttaaagcgattccagtcggcaagactcaagagaatatagacaataagcggctgttggtggaagatgaaaagcgcgcggaagactacaaaggggtgaagaagttgttggacagatactacctctcttttatcaatgatgtcttgcactcaatcaaattgaagaatctgaacaactacatctccctcttcagaaagaaaacaaggacagaaaaggagaataaggaacttgaaaatttggagatcaatctgaggaaagagatcgcgaaagcctttaaaggcaacgaaggatacaaaagtctgttcaagaaggatataattgagacaattttgccagagttcctcgatgacaaggacgagattgcgctggtcaattcgttcaacggattcacaacagcattcacaggcttctttgataatcgggaaaatatgttctctgaggaggcaaagtccacttctattgcgttcaggtgtatcaatgagaatctcactaggtacatttccaacatggatatctttgagaaggttgacgcaatttttgacaagcacgaagttcaggagattaaggagaagatcctcaattccgattatgacgttgaggacttcttcgaaggtgagttttttaatttcgtgctcactcaagagggtatcgacgtgtataatgcgatcatcggtgggttcgtgactgagtccggtgaaaagattaagggattgaacgagtatatcaacctttacaaccaaaagacgaaacagaagctgccaaagttcaagcctctttacaaacaggttctttcagaccgcgagtcactctcgttctatggggagggctacacttcggatgaggaagtcctggaggtgttcaggaatactctcaataagaattcggagattttctcttctataaaaaaactggaaaagttgtttaagaattttgacgaatactctagcgccggcatatttgtgaaaaacggcccggccatatcaacgataagtaaagatatcttcggcgaatggaacgtgatcagagacaaatggaacgcggagtatgacgatattcacctgaagaagaaggctgtcgtaacggagaagtacgaggatgatcgcaggaaaagcttcaaaaagatcggaagtttcagcctggaacagttgcaggagtatgctgacgccgatcttagcgtcgtcgagaagttgaaggagataatcatccaaaaggtcgacgagatatataaagtctatggatcaagtgaaaaactgttcgacgccgacttcgttttggagaagtccctgaagaagaacgacgctgttgttgccattatgaaggatctgctcgacagcgtgaagagtttcgagaactatattaaggcttttttcggggaggggaaggagactaacagagatgagtccttctacggagacttcgtcctcgcgtacgatatactccttaaggtagaccacatctacgacgcaatcagaaattacgtgacacaaaagccgtacagcaaggacaagttcaaactctacttccagaacccccagttcatgggcggctgggacaaggacaaggaaacggattacagggctacgatcctgaggtatggttcaaaatactacttggcgattatggacaagaagtacgccaagtgtctccagaagattgacaaagacgatgtcaatggcaattatgagaagatcaactacaagctgcttccgggtccgaacaagatgctcccaaaggttttcttcagcaagaaatggatggcctactataacccaagcgaggacatccagaagatttataagaacggtacgttcaagaagggcgacatgttcaatcttaacgactgtcacaagctgatcgacttcttcaaagactcaattagccggtacccaaagtggtctaacgcctatgacttcaacttttcggaaaccgagaagtacaaggatatagccggattttatagagaggtggaagagcagggctacaaggtgtcattcgagtccgccagcaagaaggaagtggacaagctcgtggaagagggtaagctctacatgttccagatttataataaagactttagcgataagagccacgggacacctaatctccacacaatgtatttcaagctgctcttcgacgagaataaccacggccaaatcaggttgtcaggaggggctgaactcttcatgcggcgcgctagccttaagaaggaggagcttgtagtccaccctgcgaatagtccaattgcgaataagaacccggacaatcctaaaaagactacaacattgagctacgacgtgtacaaggataagaggttttccgaggatcagtacgagctccacatcccgattgcgatcaacaagtgcccaaagaatattttcaagataaacacagaggtgcgtgtactcctgaagcatgacgacaatccttacgtcattgggattgatcggggcgagaggaacctcctctatattgtggtggtggacgggaaggggaacatagtcgaacagtactcccttaacgaaataattaacaatttcaacggcatccgtatcaagaccgactaccattcgttgctggacaagaaggagaaggagagatttgaggcgcggcaaaattggacaagtatcgagaacatcaaggaactcaaagcaggttatatctctcaagttgtgcataagatatgcgagctggttgagaagtatgacgcagtgatcgctcttgaggacctcaactcgggctttaagaattctagagttaaagtggagaagcaggtctatcaaaagttcgagaagatgcttatagataagctcaactacatggtcgataagaaatcgaacccatgtgccaccggcggcgcactcaaaggttaccaaataacaaacaaattcgagtccttcaaatcgatgagtactcagaatgggttcatattttatataccggcgtggcttacgtctaagatcgacccgtcaactggttttgtcaacctgttgaagacgaaatacacgtccattgccgattcgaaaaagttcatatctagttttgatcgtattatgtacgtcccagaggaagatcttttcgagtttgctctcgactacaaaaacttttcgcggaccgatgcggattacattaaaaaatggaaactctattcgtacggcaacagaatcaggatttttcgcaaccctaagaagaataacgtctttgattgggaggaagtttgcttgactagcgcgtacaaggagctctttaataagtatggcattaactaccaacagggtgatatcagagcactgctttgcgaacaatctgacaaggctttctactcatccttcatggctttgatgagcctgatgctccagatgagaaattcaattacaggcagaaccgacgtggatttcttgatctccccggttaaaaattctgatggcatcttttacgatagcaggaactatgaagcgcaagagaatgcgattctgccaaaaaatgcagacgccaacggtgcctataacatcgccaggaaagtcctgtgggcgatcggccagttcaaaaaggccgaagacgaaaaattggacaaggtcaaaatcgctatcagcaacaaagagtggctggagtatgctcagacatccgtaaagcataagcgtcctgctgccaccaaaaaggccggacaggctaagaaaaagaagtga

SEQ ID NO: 11 - DNA, 4272 bp, Artificial Sequence
  Nicotiana benthamiana codon-optimized SpCas9 gene sequence
atggattacaaggatcacgatggagattacaaagatcacgatatagattacaaagatgatgatgataaaatggcacctaagaagaaaagaaaggttggaattcatggtgtgcctgctgcagataagaagtacagtataggacttgatatcggtaccaactctgttggatgggctgtgatcactgatgaatataaggttcctagtaagaaattcaaggtgctcggtaacacagatagacactctattaagaagaatcttataggagctcttttgtttgattcaggtgaaacagctgaggcaaccagacttaaaaggacagcaagaaggagatacaccaggagaaagaacagaatttgttatttgcaagaaatcttctctaatgagatggctaaggttgatgattcatttttccatagattagaagagagttttcttgtggaagaggataagaaacatgaaagacaccctatattcggaaatattgttgatgaagtggcttaccatgagaaatatccaacaatctaccacttgagaaagaaactcgttgattctaccgataaagcagatctcaggttaatctaccttgctttggcacatatgataaagtttagaggacacttcttgattgagggagatcttaatcctgataactcagatgttgataagctttttattcaacttgtgcagacatataaccaacttttcgaagagaatccaatcaacgcttcaggagttgatgctaaagcaatattgagtgcaagactctctaagtctaggagactcgaaaatcttatagctcagttgcctggagaaaagaagaacggattattcggtaaccttatcgcactctctctcggtcttactccaaacttcaagtcaaacttcgatcttgctgaagatgcaaaattgcaactctctaaggatacatacgatgatgatttggataatctcttagctcagattggagatcaatatgcagatctttttcttgctgcaaaaaacctctcagatgctatccttttgagtgatatacttagagttaacactgaaattacaaaggctcctctttcagcaagtatgatcaagagatacgatgagcatcaccaggatttgactctcttaaaggctttagttagacaacagcttccagaaaagtataaggagattttctttgatcagtctaagaacggatatgctggttacatcgatggaggtgcatctcaagaagagttctacaagttcattaaacctatcttggaaaagatggatggaaccgaagagcttttggttaaactcaacagagaggatctcttaagaaagcagaggactttcgataacggatctatccctcatcaaatacaccttggtgaattgcatgctattttgaggagacaagaggatttctacccattcctcaaggataacagagaaaagattgagaagattcttacctttaggatcccttattacgttggaccattggctaggggtaacagtaggttcgcatggatgactagaaaatctgaagagacaattaccccttggaattttgaagaggttgtggataagggtgcttctgcacagtcttttattgaaagaatgacaaacttcgataagaatttgcctaacgagaaagttctcccaaagcattctcttttgtacgaatacttcactgtgtacaatgagcttacaaaggttaaatatgtgaccgaaggaatgagaaagccagcttttctttcaggagagcagaagaaagcaatcgttgatctcttattcaaaactaacagaaaggttacagtgaagcaacttaaggaagattacttcaagaaaatcgagtgcttcgattctgttgaaatatcaggagtggaggatagattcaatgcttctttgggtacttatcatgatcttttgaagattatcaaggataaggattttcttgataatgaggagaacgaagatattcttgaggatatcgttttgactctcacattattcgaagatagagagatgattgaagagaggttaaaaacatacgctcaccttttcgatgataaggttatgaaacaacttaagaggagaaggtataccggatggggtagattgtctaggaagctcatcaacggaataagagataaacagtcaggaaagactatcctcgatttcttaaagagtgatggattcgctaacagaaacttcatgcaattgatccatgatgattctctcacttttaaagaagatattcaaaaggctcaggtttcaggacagggagatagtttgcatgagcacattgctaatctcgcaggatcacctgctattaagaagggtatattgcaaactgttaaggttgtggatgaactcgttaaagtgatgggaagacataagccagagaatatagtgattgaaatggctagggagaaccaaactacacagaaaggtcaaaagaattctagagaaaggatgaaaagaatcgaagagggaattaaggagttgggttcacaaattctcaaagaacatcctgttgagaatacacaacttcagaacgaaaagctttacttgtattacttgcagaacggaagagatatgtatgtggatcaagagctcgatattaataggcttagtgattacgatgttgatcacatcgtgcctcagtcttttctcaaggatgattcaatagataacaaggttcttactagatcagataagaataggggaaagtctgataacgtgccatcagaagaggttgttaagaagatgaagaactactggagacagctcctcaacgctaagctcataactcaaagaaagttcgataatctcacaaaagctgaaaggggaggtctttctgagttggataaagcaggattcattaagagacagttggttgaaactaggcaaattacaaaacatgtggctcaaatccttgattcaaggatgaatactaagtacgatgaaaacgataagttgataagagaggttaaggttattacactcaagagtaaacttgtttctgatttcagaaaggatttccagttctacaaggtgagggagattaataactaccatcacgctcacgatgcatatcttaacgctgttgtgggaacagcattaatcaagaaataccctaagcttgaatctgagttcgtttacggagattacaaggtttacgatgtgagaaaaatgattgctaagtcagaacaagagattggtaaagctactgcaaagtactttttctatagtaacattatgaactttttcaaaaccgaaatcactttggctaacggagagatcagaaagaggccactcatagaaaccaacggagaaactggagagattgtttgggataaaggtagagatttcgctacagttaggaaggtgctttctatgcctcaggttaacatcgtgaagaaaacagaagttcaaaccggaggttttagtaaggagtctatattgccaaagagaaactcagataagctcattgctaggaagaaagattgggatcctaagaaatacggaggtttcgatagtccaacagttgcttattctgtgttggttgtggcaaaggttgaaaagggaaaaagtaagaaacttaagtctgtgaaggagcttttgggtatcactattatggaaagatcttcattcgagaaaaaccctatagatttccttgaagctaaaggatacaaggaggttaagaaagatttgataattaaactcccaaagtattcactcttcgaattagagaatggtagaaaaaggatgttagctagtgcaggagaacttcaaaagggtaacgagctcgctctcccttctaagtatgttaattttctttacttggcatctcattatgagaagcttaaaggttcaccagaagataatgagcaaaaacagcttttcgtggaacagcataagcactacttggatgaaatcatagagcaaatttcagaattttctaagagagttattttggctgatgcaaacttagataaggtgctttctgcttacaataagcatagagataagcctataagggaacaagcagagaacattatccacctttttaccttgactaatctcggagctccagctgcttttaagtacttcgataccactatcgatagaaaaaggtatacatctaccaaggaagttttggatgcaactctcattcatcagtctatcaccggtctttatgagactagaattgatctttcacaacttggaggagataaaaggccggcggccacgaaaaaggccggccaggcaaaaaagaaaaagtaa

SEQ ID NO: 12 - DNA, 27 bp, Nicotiana benthamiana/Nicotiana tobacum
  misc_feature: N.benthamiana/N. tobacum conserved crPDS1 target loci sequence
tttctgccgttaatttgagagtccaag

SEQ ID NO: 13 - DNA, 27 bp, Lycopersicon esculentum
  misc_feature: Tomato crPDS2 target loci sequence
tttctgctgttaacttgagagtccaag

SEQ ID NO: 14 - DNA, 27 bp, Capsicum annuum
  misc_feature: Pepper crPDS3 target loci sequence
tttctgctgtcaacttgagagtccaag

SEQ ID NO: 15 - DNA, 27 bp, Arachis hypogaea/Glycine max
  misc_feature: Peanut and soybean crPDS4 target loci sequence
tttgacagaaaactgaagaacacatat

SEQ ID NO: 16 - DNA, 23 bp, Nicotiana benthamiana
  misc_feature: N. benthamiana 16c gGFP target loci sequence
gatacccagatcatatgaagcgg

SEQ ID NO: 17 - DNA, 23 bp, Nicotiana benthamiana/Nicotiana tabacum
  misc_feature: N.benthamiana/N. tobacum conserved gPDS target loci sequence
ggactcttgccagcaatgcttgg

SEQ ID NO: 18 - DNA, 105 bp, Artificial Sequence
  crRNA sequence targeting crPDS1
gcccttgctcaccatactagtatctacacttagtagaaatttgccgttaatttgagagtccaagatctacacttagtagaaattactagttatggttattggtac

SEQ ID NO: 19 - DNA, 105 bp, Artificial Sequence
  crRNA sequence targeting crPDS2
gcccttgctcaccatactagtatctacacttagtagaaatttgctgttaacttgagagtccaagatctacacttagtagaaattactagttatggttattggtac

SEQ ID NO: 20 - DNA, 105 bp, Artificial Sequence
  crRNA sequence targeting crPDS3
gcccttgctcaccatactagtatctacacttagtagaaatttgctgtcaacttgagagtccaagatctacacttagtagaaattactagttatggttattggtac

SEQ ID NO: 21 - DNA, 105 bp, Artificial Sequence
  crRNA sequence targeting crPDS4
gcccttgctcaccatactagtatctacacttagtagaaattacagaaaactgaagaacacatatatctacacttagtagaaattactagttatggttattggtac

SEQ ID NO: 22 - DNA, 138 bp, Artificial Sequence
  crRNA sequence targeting gGFP
cacctgttcctgtaaggatccgatacccagatcatatgaaggttttagagctagaaatagcaagttaaaataaggctagtccgttatcaacttgaaaaagtggcaccgagtcggtgcactagttcttgccgtgtccag

SEQ ID NO: 23 - DNA, 138 bp, Artificial Sequence
  crRNA sequence targeting gPDS1
cacctgttcctgtaaggatccggactcttgccagcaatgctgttttagagctagaaatagcaagttaaaataaggctagtccgttatcaacttgaaaaagtggcaccgagtcggtgcactagttcttgccgtgtccag

SEQ ID NO: 24 - DNA, 26 bp, Artificial Sequence
  Primer NSm/F
atgttgactttttttggtaataaggg

SEQ ID NO: 25 - DNA, 27 bp, Artificial Sequence
  Primer NSm/R
ctatatttcatcaaaagataactgagc

SEQ ID NO: 26 - DNA, 27 bp, Artificial Sequence
  Primer IGR/F
tacttttaataccacttatttaagctt

SEQ ID NO: 27 - DNA, 24 bp, Artificial Sequence
  Primer M 3' UTR/R
agagcaatcagtgcaaacaaaaac

SEQ ID NO: 28 - DNA, 28 bp, Artificial Sequence
  Primer L 3'UTR/F
agagcaatcaggtaacaacgattttaag

SEQ ID NO: 29 - DNA, 25 bp, Artificial Sequence
  Primer M 3'UTR/F
agagcaatcagtgcaaacaaaaacc

SEQ ID NO: 30 - DNA, 29 bp, Artificial Sequence
  Primer S 3'UTR/F
agagcaattgtgtcaattttattcaaacc

SEQ ID NO: 31 - DNA, 57 bp, Artificial Sequence
  Primer L(+)/F
atataaggaagttcatttcatttggagaggagagcaatcaggtaacaacgattttaa

SEQ ID NO: 32 - DNA, 54 bp, Artificial Sequence
  32 Primer L(+)/R
cgcgaggaggtggagatgccatgccgacccagagcaatcaggtacaactaaaac

SEQ ID NO: 33 - DNA, 54 bp, Artificial Sequence
  Primer Lopt 5'UTR/F
gattctgatgaggaagaggacaccgattagattaaaagtaatgcctaacaatgc

SEQ ID NO: 34 - DNA, 54 bp, Artificial Sequence
  Primer Lopt 3'UTR/R
caatcagcttctggattttctggatgttcatgtttgcttaaaatcgttgttacc

SEQ ID NO: 35 - DNA, 34 bp, Artificial Sequence
  Primer M 5'UTR/F
tttcatttggagaggagagcaatcagtgcatcag

SEQ ID NO: 36 - DNA, 40 bp, Artificial Sequence
  Primer M 3'UTR/R
atgccatgccgacccagagcaatcagtgcaaacaaaaacc

SEQ ID NO: 37 - DNA, 29 bp, Artificial Sequence
  Primer M IGR/ScaI/F
ttgatgaaatatagtacttttaataccac

SEQ ID NO: 38 - DNA, 33 bp, Artificial Sequence
  Primer M IGR/R
cacctgttcctgtaaggctgcttgtcacaagct

SEQ ID NO: 39 - DNA, 20 bp, Artificial Sequence
  Primer RFP/F
tggcctcctccgagaacgtc

SEQ ID NO: 40 - DNA, 20 bp, Artificial Sequence
  Primer RFP/F
ttacaggaacaggtggtggc

SEQ ID NO: 41 - DNA, 42 bp, Artificial Sequence
  Primer RFP/M 3'UTR/F
ctcggaggaggccatcttatacgtctgctcagattataatgg

SEQ ID NO: 42 - DNA, 26 bp, Artificial Sequence
  Primer pCB-PmeI/R
aaacactgatagtttaaactgaaggc

SEQ ID NO: 43 - DNA, 39 bp, Artificial Sequence
  Primer 35S/M 3'UTR/F
tttcatttggagaggagagcaatcagtgcaaacaaaaac

SEQ ID NO: 44 - DNA, 34 bp, Artificial Sequence
  Primer HDV/M 5'UTR/R
atgccatgccgacccagagcaatcagtgcatcag

SEQ ID NO: 45 - DNA, 43 bp, Artificial Sequence
  Primer 35S/S 3'UTR/F
tttcatttggagagggagcaattgtgtcaattttattcaaacc

SEQ ID NO: 46 - DNA, 41 bp, Artificial Sequence
  Primer HDV/S 5'UTR/R
atgccatgccgacccagagcaattgtgtcataattttattc

SEQ ID NO: 47 - DNA, 22 bp, Artificial Sequence
  Primer S 5'UTR/F
tatggttattggtactgtgttc

SEQ ID NO: 48 - DNA, 21 bp, Artificial Sequence
  Primer S IGR/R
tcttgccgtgtccagcttttc

SEQ ID NO: 49 - DNA, 31 bp, Artificial Sequence
  Primer GFP/5'UTR/F
gtaccaataaccataatggtgagcaagggcg

SEQ ID NO: 50 - DNA, 37 bp, Artificial Sequence
  Primer GFP/IGR/R
ctggacacggcaagattacttgtacagctcgtccatg

SEQ ID NO: 51 - DNA, 40 bp, Artificial Sequence
  Primer BamHI/NSs/F
atctatctctggatccatgtcttcaagtgtttatgagtcg

SEQ ID NO: 52 - DNA, 40 bp, Artificial Sequence
  Primer SalI/NSs/R
aacgagctctgtcgacttattttgatcctgaagcatatgc

SEQ ID NO: 53 - DNA, 38 bp, Artificial Sequence
  Primer BamHI/NSm/F
atctctggatccatgttgactttttttggtaataaggg

SEQ ID NO: 54 - DNA, 41 bp, Artificial Sequence
  Primer SalI/NSm/R
cgagctctgtcgacctatatttcatcaaaagataactgagc

SEQ ID NO: 55 - DNA, 43 bp, Artificial Sequence
  Primer M UTR/Cas12a/F
gagcagacgtataagatggattacaaggatgacgacgataaga

SEQ ID NO: 56 - DNA, 25 bp, Artificial Sequence
  Primer Cas12a/R
tcacttctttttcttagcctgtccg

SEQ ID NO: 57 - DNA, 40 bp, Artificial Sequence
  Primer Cas12a/M IGR/R
aagaaaaagaagtgaggctgcttgtcacaagctaaatttg

SEQ ID NO: 58 - DNA, 25 bp, Artificial Sequence
  Primer SpeI/GFP/F
actagtatggtgagcaagggcgagg

SEQ ID NO: 59 - DNA, 25 bp, Artificial Sequence
  Primer IGR PacI/R
ataagtgtgtttaattaaagtttgc

SEQ ID NO: 60 - DNA, 21 bp, Artificial Sequence
  Primer NOS Pvu1/F
ccaaatgtttgaacgatcggg

SEQ ID NO: 61 - DNA, 35 bp, Artificial Sequence
  Primer 5'UTR/R
actagttatggttattggtactgtgttcttattac

SEQ ID NO: 62 - DNA, 39 bp, Artificial Sequence
  Primer S UTR/RFP/F
gtaccaataaccataggatcatggcctcctccgagaacg

SEQ ID NO: 63 - DNA, 43 bp, Artificial Sequence
  Primer Cas9/F
gagcagacgtataagggatccatggattacaaggatcacgatg

SEQ ID NO: 64 - DNA, 39 bp, Artificial Sequence
  Primer Cas9/R
caagcagccgtcgacttactttttcttttttgcctggcc

SEQ ID NO: 65 - DNA, 27 bp, Artificial Sequence
  Primer M 3'UTR/F
cttatacgtctgctcagattataatgg

SEQ ID NO: 66 - DNA, 31 bp, Artificial Sequence
  Primer Cas9/M IGR/R
gtcgacggctgcttgtcacaagctaaatttg

SEQ ID NO: 67 - DNA, 39 bp, Artificial Sequence
  Primer gPDS1/NSs/F
caagagtccggatccttattttgatcctgaagcatatgc

SEQ ID NO: 68 - DNA, 26 bp, Artificial Sequence
  Primer gPDS1/F
ggatccggactcttgccagcaatgct

SEQ ID NO: 69 - DNA, 39 bp, Artificial Sequence
  Primer IGR/scaffold/R
ctggacacggcaagaactagtgcaccgactcggtgccac

SEQ ID NO: 70 - DNA, 23 bp, Artificial Sequence
  Primer crPDS1 forward primer
taaaatgccccaaattggacttg

SEQ ID NO: 71 - DNA, 26 bp, Artificial Sequence
  Primer crPDS1 reverse primer
gctactaccaaaacataacaaattcc

SEQ ID NO: 72 - DNA, 22 bp, Artificial Sequence
  Primer crPDS2 forward primer
gaggtttgtggatcttttaggc

SEQ ID NO: 73 - DNA, 22 bp, Artificial Sequence
  Primer crPDS2 reverse primer
ccagcaaaacataacgaattcc

SEQ ID NO: 74 - DNA, 23 bp, Artificial Sequence
  Primer crPDS3 forward primer
gccttcggttcaatttgtttgtc

SEQ ID NO: 75 - DNA, 23 bp, Artificial Sequence
  Primer crPDS3 reverse primer
gtcactaccaccaaaacataacg

SEQ ID NO: 76 - DNA, 21 bp, Artificial Sequence
  crPDS4 forward primer
ttgagaagtgaaactgtgaag

SEQ ID NO: 77 - DNA, 22 bp, Artificial Sequence
  crPDS4 reverse primer
tgtgaggcacaaagttataagc

SEQ ID NO: 78 - DNA, 26 bp, Artificial Sequence
  crPDS4 forward primer
atggttgtaatagttttggtaaatgg

SEQ ID NO: 79 - DNA, 22 bp, Artificial Sequence
  crPDS4 reverse primer
agggagaggatatcttctacac

SEQ ID NO: 80 - DNA, 26 bp, Artificial Sequence
  gGFP1 forward primer
atgagtaaaggagaagaacttttcac

SEQ ID NO: 81 - DNA, 24 bp, Artificial Sequence
  gGFP1 reverse primer
ttatttgtatagttcatccatgcc

SEQ ID NO: 82 - DNA, 26 bp, Artificial Sequence
  gPDS1 forward primer
atgcgttattacttctacaggaattt

SEQ ID NO: 83 - DNA, 21 bp, Artificial Sequence
  gPDS1 reverse primer
acttgctttctcatccagtcc

SEQ ID NO: 84 - DNA, 4914 bp, Artificial Sequence
  Codon-optimized ABE sequence
atggattacaaggaccacgacggtgattataaggatcacgacatcgactacaaggacgatgatgacaagatggctccgaagaagaaaaggaaagtgtctgaagtagagttctcccacgagtactggatgaggcacgctcttacattggccaagcgtgctagggacgagagagaggtgcctgtcggagctgtgcttgtactgaacaaccgagtaatcggcgaaggctggaaccgtgccattggtctgcatgatcccaccgcacacgcagagatcatggcacttcgtcaaggaggtcttgtaatgcagaactaccgtctgatagatgcaactctctacgtgaccttcgagccctgtgtcatgtgtgctggagcaatgatccactcccgtatcggtcgagtggtattcggctggcgtaacagcaagagaggtgctgctggtagcctcatgaacgtgctgaactaccctggtatgaaccatcgtgtagagatcactgagggcattcttgcagacgagtgtgctgcactgctctgcgacttctacaggatgcctaggcaggtgttcaatgctcagaagaaggctcagagctccatcaatagcggtggatcctcaggtggatcttcaggcagtgagacacctggaaccagtgagtcagctactccagagtcaagtggtggatcttcaggaggctcaatacacggtgttccagcagccgataagaagtacagtatcggacttgccatagggactaactctgtcgggtgggcagtaatcacagatgagtacaaagtcccatctaagaagttcaaggtgctcggtaacaccgatagacacagcatcaagaagaacctcatcggtgctctcctgttcgattccggcgaaacggccgaagccactaggttgaagaggacggcccgacgacgttatacccgtagaaagaataggatatgctatctgcaggagatattctccaacgagatggctaaggtagacgatagcttcttccatcgtctcgaggagtccttcctggtggaagaggacaagaaacatgaaagacacccaatctttgggaacattgttgacgaggtcgcatatcatgagaagtacccaacaatctaccacttgaggaagaaactcgtcgacagtactgacaaggctgatctgcgtttaatctacttagcactggctcatatgatcaagttcagaggtcacttcttgatcgagggtgacttgaaccctgacaattcagacgtagacaagctgttcatccagttagtccagacgtataatcagttgttcgaggaaaacccaattaacgctagtggagtcgacgccaaggcaatattgagtgcaagactctccaagtcccgaaggttggaaaacctcattgctcaattgcctggagagaagaagaacgggctcttcggaaatcttatagctctgtccttagggttaacgccgaatttcaagtccaacttcgacctcgccgaggacgccaagttgcaattgtccaaggatacctacgacgatgacctcgacaacttactggctcagatcggcgaccagtacgctgacctcttcttggccgctaagaacttgtcagacgcaatcctcttaagtgatatcttacgtgtgaacacagagattacgaaagctcctttgagcgcatccatgatcaagagatacgatgagcaccatcaggatttgacgttgttgaaggccttagttcgtcagcaattgcccgagaagtacaaggagatcttcttcgatcagtccaagaacggatacgcagggtacatcgatggtggtgctagtcaagaggagttttacaagttcatcaagcccatactcgagaagatggatggaactgaggaactgttagtgaagctgaatcgtgaggacctgttaaggaagcagcgaacgttcgacaatggcagcatcccgcaccagatccaccttggcgagctgcatgcaatcttgaggagacaggaagacttctatccattcttgaaggacaacagagagaagatcgagaagatcttgacgttcagaatcccgtattacgttggtccactcgccaggggtaactcccgtttcgcttggatgacgaggaaatcagaggagacaatcactccttggaacttcgaggaggtggttgacaaaggagccagcgctcaatccttcatagagcgtatgaccaatttcgacaagaatctcccaaacgagaaggtcctgccgaaacactcattgttgtacgagtacttcactgtgtataacgagctcacgaaggtcaaatacgtaactgagggtatgcgaaagcccgccttcctctccggtgaacagaagaaggcaatcgtcgatttgttgttcaagaccaacaggaaggtcactgtgaagcaactgaaagaggactacttcaagaagatagagtgcttcgattctgtggagatcagtggtgttgaggatcgtttcaacgcatccttgggcacataccatgatttgttgaagatcatcaaggacaaggacttcctcgacaacgaggagaacgaggacatcctcgaggatatcgttctcacattgacgctcttcgaggatcgtgagatgatcgaggagagactgaagacctacgctcatttgttcgatgataaggtgatgaagcaactcaagaggcgtcgatacacgggatggggaaggttgtctcggaagctgatcaacggtattagggataaacagtctggcaagacaatcttggacttcttgaagagtgatggattcgcaaataggaatttcatgcagttaatccacgatgatagtctgacgttcaaggaggacatccaaaaggcccaagtgagtggtcagggagacagcctccatgaacatatagcaaacttggctggatccccagcaattaagaaaggaatcttgcagacggtcaaagttgtggatgaacttgttaaggtcatgggtcgtcacaaacctgagaatatcgttatcgaaatggcccgagagaatcagacgacccagaaaggacagaagaactctcgtgaacgtatgaaacgaatagaagaagggatcaaagagctcggtagccagatcctgaaggagcacccagtagagaacactcaactgcagaacgagaagctgtatctgtactacttgcaaaacgggcgagatatgtatgttgaccaggagctcgacatcaatagactttctgactacgatgttgaccatattgtgccgcaaagcttcttgaaggatgatagcatagataacaaagttctcacacgttccgacaagaacagaggtaagagcgacaacgtgccgagtgaagaagtcgttaagaagatgaagaactactggaggcagttgctcaacgctaagttgatcacccagaggaagttcgacaacctcacaaaggctgagagaggaggcctgtcagagttggataaggctgggttcatcaagaggcagcttgtcgagacacgacagatcaccaagcacgtagcccagatcctcgattcaaggatgaacaccaagtacgatgagaacgacaagctcatcagggaagtgaaggtaatcacgctgaagagcaagctcgtatccgacttccgaaaggactttcagttctacaaggtgcgtgagatcaacaactaccaccatgctcatgatgcatatcttaatgcagtggttgggacggctctcattaagaagtacccaaagctcgaatctgaatttgtgtatggcgattacaaggtttatgatgtccgtaagatgattgctaagagcgagcaggagattggtaaggctaccgcgaagtacttcttctactctaacatcatgaacttcttcaagacggagatcaccctggccaacggagagatcaggaagcgtccgctcatcgagaccaacggtgagaccggtgagatcgtgtgggacaagggacgtgacttcgccactgtgaggaaggtgttgagcatgccgcaggtgaacatcgtgaagaagacggaggtgcagaccggagggttctccaaggaatcaatcttgccaaagaggaactccgataaactcatagcaaggaagaaggattgggatcccaagaagtatggagggttcgactccccgaccgtcgcctacagcgtcttggttgtggcaaaggtggagaagggaaagagcaagaagttgaaatcagtcaaggagctccttggaatcacaatcatggagcgaagttctttcgagaagaaccccatagacttcttggaggccaaaggttacaaagaagtgaagaaagacttgataatcaagttgcctaagtactccttgttcgagctcgagaacgggaggaagcgaatgttggccagcgccggagaacttcagaaaggcaacgagctcgctctcccaagcaagtacgtgaatttcttgtacctcgcatcacactacgagaagctgaagggcagcccggaggataacgaacagaagcagctcttcgtggagcaacacaagcactacttggatgagatcatcgagcagattagcgagttcagcaagagggtaatcttggctgacgctaatctggacaaggttctcagcgcatacaacaagcatcgtgacaaacccatccgagagcaggcagagaacatcatccacttgttcaccctgactaatttgggagcacccgcagccttcaagtacttcgatactaccatcgaccggaagagatacacaagtaccaaggaggtcctggatgcaaccttgatccatcagtccatcaccggcttgtacgagactaggatcgacctctctcagttgggtggagactccggcggcagcccaaagaagaagcggaaggtgtctggaggttctcctaagaaaaagagaaaagtgtccggcggctccccgaagaagaagcgcaaggtgtag

SEQ ID NO: 85 - DNA, 5175 bp, Artificial Sequence
  Codon-optimized CBE sequence
atggattacaaggaccacgacggtgattataaggatcacgacatcgactacaaggacgatgatgacaagatggctccgaagaagaaaaggaaagtgggtatacgagaagcctctccagcatctggtcccaggcatctgatggatccacacatcttcacatccaacttcaacaacggcatcggacgacacaagacgtatctgtgctacgaggtagagaggttggacaacgggacttcagtgaagatggaccagcacagaggcttcttgcacaaccaagccaagaacttgctgtgcggattctacgggaggcatgccgagttaagattcctcgacttggttccaagcttgcagctcgacccggcacagatctatcgagtcacgtggttcatcagttggtccccgtgcttcagttggggatgtgcaggtgaggtgagagcattcctgcaggagaacactcatgtccgattgcgtatcttcgcagcccgaatctacgactacgacccattgtacaaagaggcactgcagatgctcagggacgccggtgcacaggtctccatcatgacatacgacgagttcaagcactgttgggacacattcgtcgatcatcaaggttgcccattccagccttgggacggtttggacgaacacagccaggctctctctggaaggctgagggccattcttcagaaccagggcaactcaggatctgaaacgccgggtaccagtgaaagtgccacacccgagagtatacacggtgttccagcagccgataagaagtacagtatcggacttgccatagggactaactctgtcgggtgggcagtaatcacagatgagtacaaagtcccatctaagaagttcaaggtgctcggtaacaccgatagacacagcatcaagaagaacctcatcggtgctctcctgttcgattccggcgaaacggccgaagccactaggttgaagaggacggcccgacgacgttatacccgtagaaagaataggatatgctatctgcaggagatattctccaacgagatggctaaggtagacgatagcttcttccatcgtctcgaggagtccttcctggtggaagaggacaagaaacatgaaagacacccaatctttgggaacattgttgacgaggtcgcatatcatgagaagtacccaacaatctaccacttgaggaagaaactcgtcgacagtactgacaaggctgatctgcgtttaatctacttagcactggctcatatgatcaagttcagaggtcacttcttgatcgagggtgacttgaaccctgacaattcagacgtagacaagctgttcatccagttagtccagacgtataatcagttgttcgaggaaaacccaattaacgctagtggagtcgacgccaaggcaatattgagtgcaagactctccaagtcccgaaggttggaaaacctcattgctcaattgcctggagagaagaagaacgggctcttcggaaatcttatagctctgtccttagggttaacgccgaatttcaagtccaacttcgacctcgccgaggacgccaagttgcaattgtccaaggatacctacgacgatgacctcgacaacttactggctcagatcggcgaccagtacgctgacctcttcttggccgctaagaacttgtcagacgcaatcctcttaagtgatatcttacgtgtgaacacagagattacgaaagctcctttgagcgcatccatgatcaagagatacgatgagcaccatcaggatttgacgttgttgaaggccttagttcgtcagcaattgcccgagaagtacaaggagatcttcttcgatcagtccaagaacggatacgcagggtacatcgatggtggtgctagtcaagaggagttttacaagttcatcaagcccatactcgagaagatggatggaactgaggaactgttagtgaagctgaatcgtgaggacctgttaaggaagcagcgaacgttcgacaatggcagcatcccgcaccagatccaccttggcgagctgcatgcaatcttgaggagacaggaagacttctatccattcttgaaggacaacagagagaagatcgagaagatcttgacgttcagaatcccgtattacgttggtccactcgccaggggtaactcccgtttcgcttggatgacgaggaaatcagaggagacaatcactccttggaacttcgaggaggtggttgacaaaggagccagcgctcaatccttcatagagcgtatgaccaatttcgacaagaatctcccaaacgagaaggtcctgccgaaacactcattgttgtacgagtacttcactgtgtataacgagctcacgaaggtcaaatacgtaactgagggtatgcgaaagcccgccttcctctccggtgaacagaagaaggcaatcgtcgatttgttgttcaagaccaacaggaaggtcactgtgaagcaactgaaagaggactacttcaagaagatagagtgcttcgattctgtggagatcagtggtgttgaggatcgtttcaacgcatccttgggcacataccatgatttgttgaagatcatcaaggacaaggacttcctcgacaacgaggagaacgaggacatcctcgaggatatcgttctcacattgacgctcttcgaggatcgtgagatgatcgaggagagactgaagacctacgctcatttgttcgatgataaggtgatgaagcaactcaagaggcgtcgatacacgggatggggaaggttgtctcggaagctgatcaacggtattagggataaacagtctggcaagacaatcttggacttcttgaagagtgatggattcgcaaataggaatttcatgcagttaatccacgatgatagtctgacgttcaaggaggacatccaaaaggcccaagtgagtggtcagggagacagcctccatgaacatatagcaaacttggctggatccccagcaattaagaaaggaatcttgcagacggtcaaagttgtggatgaacttgttaaggtcatgggtcgtcacaaacctgagaatatcgttatcgaaatggcccgagagaatcagacgacccagaaaggacagaagaactctcgtgaacgtatgaaacgaatagaagaagggatcaaagagctcggtagccagatcctgaaggagcacccagtagagaacactcaactgcagaacgagaagctgtatctgtactacttgcaaaacgggcgagatatgtatgttgaccaggagctcgacatcaatagactttctgactacgatgttgaccatattgtgccgcaaagcttcttgaaggatgatagcatagataacaaagttctcacacgttccgacaagaacagaggtaagagcgacaacgtgccgagtgaagaagtcgttaagaagatgaagaactactggaggcagttgctcaacgctaagttgatcacccagaggaagttcgacaacctcacaaaggctgagagaggaggcctgtcagagttggataaggctgggttcatcaagaggcagcttgtcgagacacgacagatcaccaagcacgtagcccagatcctcgattcaaggatgaacaccaagtacgatgagaacgacaagctcatcagggaagtgaaggtaatcacgctgaagagcaagctcgtatccgacttccgaaaggactttcagttctacaaggtgcgtgagatcaacaactaccaccatgctcatgatgcatatcttaatgcagtggttgggacggctctcattaagaagtacccaaagctcgaatctgaatttgtgtatggcgattacaaggtttatgatgtccgtaagatgattgctaagagcgagcaggagattggtaaggctaccgcgaagtacttcttctactctaacatcatgaacttcttcaagacggagatcaccctggccaacggagagatcaggaagcgtccgctcatcgagaccaacggtgagaccggtgagatcgtgtgggacaagggacgtgacttcgccactgtgaggaaggtgttgagcatgccgcaggtgaacatcgtgaagaagacggaggtgcagaccggagggttctccaaggaatcaatcttgccaaagaggaactccgataaactcatagcaaggaagaaggattgggatcccaagaagtatggagggttcgactccccgaccgtcgcctacagcgtcttggttgtggcaaaggtggagaagggaaagagcaagaagttgaaatcagtcaaggagctccttggaatcacaatcatggagcgaagttctttcgagaagaaccccatagacttcttggaggccaaaggttacaaagaagtgaagaaagacttgataatcaagttgcctaagtactccttgttcgagctcgagaacgggaggaagcgaatgttggccagcgccggagaacttcagaaaggcaacgagctcgctctcccaagcaagtacgtgaatttcttgtacctcgcatcacactacgagaagctgaagggcagcccggaggataacgaacagaagcagctcttcgtggagcaacacaagcactacttggatgagatcatcgagcagattagcgagttcagcaagagggtaatcttggctgacgctaatctggacaaggttctcagcgcatacaacaagcatcgtgacaaacccatccgagagcaggcagagaacatcatccacttgttcaccctgactaatttgggagcacccgcagccttcaagtacttcgatactaccatcgaccggaagagatacacaagtaccaaggaggtcctggatgcaaccttgatccatcagtccatcaccggcttgtacgagactaggatcgacctctctcagttgggtggagacactagagactccggaggcagcacaaacctcagcgacatcatcgagaaggagacaggcaagcagttggtcatccaggagtctatcctcatgctgcccgaggaggttgaggaggtcattggcaataagcctgagagcgacatacttgtgcacaccgcatatgacgaatccacagatgagaatgtgatgcttctgacatcagatgcacctgagtacaagccatgggccctcgtgatccaggactcaaacggtgagaacaagatcaagatgttgagcggcgggtcgcctaagaagaagcgtaaagtgtaa

SEQ ID NO: 86 - DNA, 27 bp, Artificial Sequence
  N. benthamiana crFucT target site sequence
tttggaacagattccaataagaagcct

SEQ ID NO: 87 - DNA, 27 bp, Artificial Sequence
  N. benthamiana crDCL2 target site sequence
tttgagaagctatgcttatcttcttcg

SEQ ID NO: 88 - DNA, 27 bp, Artificial Sequence
  Ground cherry crER target site sequence
tttaatgttaaacctttagtgtccttt

SEQ ID NO: 89 - DNA, 23 bp, Artificial Sequence
  N. benthamiana gPDS2 target site sequence
ttggtagtagcgactccatgggg

SEQ ID NO: 90 - DNA, 23 bp, Artificial Sequence
  N. benthamiana gRDR6 target site sequence
cccctcctgactcttacccaact

SEQ ID NO: 91 - DNA, 23 bp, Artificial Sequence
  N. benthamiana gSGS3 target site sequence
acaagagtggaagcagtgctggg

SEQ ID NO: 92 - DNA, 23 bp, Artificial Sequence
  N. benthamiana gPDSa target site sequence
tgcaaattgagttgggagtgagg

SEQ ID NO: 93 - DNA, 23 bp, Artificial Sequence
  N. benthamiana gFucTa1 target site sequence
cctcttgagaatgttgctattgg

SEQ ID NO: 94 - DNA, 23 bp, Artificial Sequence
  N. benthamiana gFucTa2 target site sequence
cacaccttcctccaggagatagg

SEQ ID NO: 95 - DNA, 23 bp, Artificial Sequence
  N. benthamiana gRDR6a1 target site sequence
ccaatatctaggcgtgagggatt

SEQ ID NO: 96 - DNA, 23 bp, Artificial Sequence
  N. benthamiana gRDR6a2 target site sequence
cccgacttcatggggaaggagga

SEQ ID NO: 97 - DNA, 23 bp, Artificial Sequence
  N. benthamiana gBBLd target site sequence
gaaatcagagtaaggtgcggagg

SEQ ID NO: 98 - DNA, 27 bp, Artificial Sequence
  Peanut crPDS5 target site sequence
aatgcaatgtatattgattgccttaaa

SEQ ID NO: 99 - DNA, 27 bp, Artificial Sequence
  Pepper crPDS6 target site sequence
tttctgctgtcaacttgagagtccaag

SEQ ID NO: 100 - DNA, 22 bp, Artificial Sequence
  crFucT1 forward primer
ctgactttatgaatgtcccatc

SEQ ID NO: 101 - DNA, 21 bp, Artificial Sequence
  crFucT1 reverse primer
gcatagtattgagctgactcc

SEQ ID NO: 102 - DNA, 20 bp, Artificial Sequence
  crDCL2 forward primer
agttagaggcattggagacg

SEQ ID NO: 103 - DNA, 19 bp, Artificial Sequence
  crDCL2 reverse primer
ctgagccaccagaacaacc

SEQ ID NO: 104 - DNA, 22 bp, Artificial Sequence
  crER forward primer
gttcttgagctttggtcctgtg

SEQ ID NO: 105 - DNA, 20 bp, Artificial Sequence
  crER reverse primer
aatgacaactacaaacgtgg

SEQ ID NO: 106 - DNA, 20 bp, Artificial Sequence
  gPDS2 forward primer
gcttatctttggagctcgag

SEQ ID NO: 107 - DNA, 24 bp, Artificial Sequence
  gPDS2 reverse primer
cgcattcaaaacaaacctttaaag

SEQ ID NO: 108 - DNA, 20 bp, Artificial Sequence
  gRDR6 forward primer
tgggtttgacaatgatgtca

SEQ ID NO: 109 - DNA, 20 bp, Artificial Sequence
  gRDR6 reverse primer
gcatgaggtaccactttttc

SEQ ID NO: 110 - DNA, 20 bp, Artificial Sequence
  gSGS3 forward primer
cagcaaagcagaaagctatc

SEQ ID NO: 111 - DNA, 20 bp, Artificial Sequence
  gSGS3 reverse primer
atctggatgaccccaagctt

SEQ ID NO: 112 - DNA, 21 bp, Artificial Sequence
  gPDSa forward primer
gggacatttttggagtgtagc

SEQ ID NO: 113 - DNA, 20 bp, Artificial Sequence
  gPDSa reverse primer
agagttaagagtgggaactg

SEQ ID NO: 114 - DNA, 20 bp, Artificial Sequence
  gFucTa1 forward primer
caaccctcgatcacattcac

SEQ ID NO: 115 - DNA, 21 bp, Artificial Sequence
  gFucTa1 reverse primer
acacacacacactaacactag

SEQ ID NO: 116 - DNA, 21 bp, Artificial Sequence
  gFucTa2 forward primer
tggtgcatcttctaagtagcg

SEQ ID NO: 117 - DNA, 21 bp, Artificial Sequence
  gFucTa2 reverse primer
actaaaaaaaccacgacatgc

SEQ ID NO: 118 - DNA, 20 bp, Artificial Sequence
  gRDR6a1 forward primer
taggtcccaatgtccattct

SEQ ID NO: 119 - DNA, 20 bp, Artificial Sequence
  gRDR6a1 reverse primer
agctaaggattgaccgactc

SEQ ID NO: 120 - DNA, 20 bp, Artificial Sequence
  gRDR6a2 forward primer
gcagagcttgctgctctagc

SEQ ID NO: 121 - DNA, 20 bp, Artificial Sequence
  gRDR6a2 reverse primer
ccctctgtatcacatacatc

SEQ ID NO: 122 - DNA, 22 bp, Artificial Sequence
  gBBL  forward primer
agccaactgttattattgtacc

SEQ ID NO: 123 - DNA, 20 bp, Artificial Sequence
  gBBL reverse primer
aactgttgggcaagaaccag

SEQ ID NO: 124 - DNA, 41 bp, Artificial Sequence
  SpeI/Flag/F primer
gagcagacgtataagactagtatggattacaaggaccacga

SEQ ID NO: 125 - DNA, 34 bp, Artificial Sequence
  ABE/R primer
gcagccgtcgacgcgtagctcctacaccttgcgc

SEQ ID NO: 126 - DNA, 39 bp, Artificial Sequence
  CBE/R primer
gcagccgtcgacgcgttacactttacgcttcttcttagg

SEQ ID NO: 127 - DNA, 21 bp, Artificial Sequence
  crPDS5 forward primer
tatcctcatggcaggtttgac

SEQ ID NO: 128 - DNA, 22 bp, Artificial Sequence
  crPDS5 reverse primer
ccaccaaaacataacgaattcc

SEQ ID NO: 129 - DNA, 22 bp, Artificial Sequence
  crPDS6 forward primer
ccaccaaaacataacgaattcc

SEQ ID NO: 130 - DNA, 21 bp, Artificial Sequence
  crPDS6 reverse primer
gtgagcttgtcaaatttatac

SEQ ID NO: 131 - DNA, 24 bp, Artificial Sequence
  N/F primer
ctatggattacctcttgatgatgc

SEQ ID NO: 132 - DNA, 23 bp, Artificial Sequence
  N/R primer
ttaagcaagttctgcaagttttg

SEQ ID NO: 133 - DNA, 26 bp, Artificial Sequence
  Actin/F primer
caatccagacacctgtactttctctc

SEQ ID NO: 134 - DNA, 24 bp, Artificial Sequence
  Actin/R primer
aagctgcaggtatccatgagacta

SEQ ID NO: 135 - DNA, 118 bp, Artificial Sequence
  Synthesized crPDS1&Fuc sequence
actagtaatttctactaagtgtagatgaacagattccaataagaagcctaatttctactaagtgtagattgccgttaatttgagagtccaagaatttctactaagtgtagatactagt

SEQ ID NO: 136 - DNA, 161 bp, Artificial Sequence
  Synthesized crPDS1&FucT&DCL2 sequence
actagtaatttctactaagtgtagatagaagctatgcttatcttcttcgaatttctactaagtgtagatgaacagattccaataagaagcctaatttctactaagtgtagattgccgttaatttgagagtccaagaatttctactaagtgtagatactagt

SEQ ID NO: 137 - DNA, 210 bp, Artificial Sequence
  Synthesized sgNbPDS2&RDR6 sequence
actagtagttgggtaagagtcaggaggttttagagctagaaatagcaagttaaaataaggctagtccgttatcaacttgaaaaagtggcaccgagtcggtgcggatccttggtagtagcgactccatggttttagagctagaaatagcaagttaaaataaggctagtccgttatcaacttgaaaaagtggcaccgagtcggtgcactagt

SEQ ID NO: 138 - DNA, 312 bp, Artificial Sequence
  Synthesized sgNbPDS2&RDR6&SGS3-1 sequence
actagtagttgggtaagagtcaggaggttttagagctagaaatagcaagttaaaataaggctagtccgttatcaacttgaaaaagtggcaccgagtcggtgcggatccacaagagtggaagcagtgctgttttagagctagaaatagcaagttaaaataaggctagtccgttatcaacttgaaaaagtggcaccgagtcggtgcggatccttggtagtagcgactccatggttttagagctagaaatagcaagttaaaataaggctagtccgttatcaacttgaaaaagtggcaccgagtcggtgcactagt